European Patent Specification EP 3 864 152 B1, published August 16, 2023. Title: Methods and Compositions for Editing RNAs. Applicant: Peking University EdiGene Inc. The sequence listing filed with the application follows.

SEQUENCE LISTING (343 sequences)

SEQ ID NO: 1 - DNA, 708 bp, Artificial Sequence
atggtgagcaagggcgaggaggataacatggccatcatcaaggagttcatgcgcttcaaggtgcacatggagggctccgtgaacggccacgagttcgagatcgagggcgagggcgagggccgcccctacgagggcacccagaccgccaagctgaaggtgaccaagggtggccccctgcccttcgcctgggacatcctgtcccctcagttcatgtacggctccaaggcctacgtgaagcaccccgccgacatccccgactacttgaagctgtccttccccgagggcttcaagtgggagcgcgtgatgaacttcgaggacggcggcgtggtgaccgtgacccaggactcctccctgcaggacggcgagttcatctacaaggtgaagctgcgcggcaccaacttcccctccgacggccccgtaatgcagaagaagaccatgggctgggaggcctcctccgagcggatgtaccccgaggacggcgccctgaagggcgagatcaagcagaggctgaagctgaaggacggcggccactacgacgctgaggtcaagaccacctacaaggccaagaagcccgtgcagctgcccggcgcctacaacgtcaacatcaagttggacatcacctcccacaacgaggactacaccatcgtggaacagtacgaacgcgccgagggccgccactccaccggcggcatggacgagctgtacaag

SEQ ID NO: 2 - DNA, 99 bp, Artificial Sequence
ctgcagggcggaggaggcagcggcggaggaggcagcggcggaggaggcagcagaaggtatacacgccggaagaatctgtagagatccccggtcgccacc

SEQ ID NO: 3 - DNA, 717 bp, Artificial Sequence
gtgagcaagggcgaggagctgttcaccggggtggtgcccatcctggtcgagctggacggcgacgtaaacggccacaagttcagcgtgtccggcgagggcgagggcgatgccacctacggcaagctgaccctgaagttcatctgcaccaccggcaagctgcccgtgccctggcccaccctcgtgaccaccctgacctacggcgtgcagtgcttcagccgctaccccgaccacatgaagcagcacgacttcttcaagtccgccatgcccgaaggctacgtccaggagcgcaccatcttcttcaaggacgacggcaactacaagacccgcgccgaggtgaagttcgagggcgacaccctggtgaaccgcatcgagctgaagggcatcgacttcaaggaggacggcaacatcctggggcacaagctggagtacaactacaacagccacaacgtctatatcatggccgacaagcagaagaacggcatcaaggtgaacttcaagatccgccacaacatcgaggacggcagcgtgcagctcgccgaccactaccagcagaacacccccatcggcgacggccccgtgctgctgcccgacaaccactacctgagcacccagtccgccctgagcaaagaccccaacgagaagcgcgatcacatggtcctgctggagttcgtgaccgccgccgggatcactctcggcatggacgagctgtacaagtaa

SEQ ID NO: 4 - DNA, 81 bp, Artificial Sequence
ctgcagggcggaggaggcagcggcggaggaggcagcggcggaggaggcagcgcctgctcgcgatgctagagggctctgcca

SEQ ID NO: 5 - DNA, 50 bp, Artificial Sequence
ctgcagggcggaggaggcagcgcctgctcgcgatgctagagggctctgcc

SEQ ID NO: 6 - RNA, 101 nt, Artificial Sequence
ggaccaccccaaaaaugaauauaaccaaaacugaacagcuccucgcccuugcucacuggcagagcccuccagcaucgcgagcaggcgcugccuccuccgcc

SEQ ID NO: 7 - RNA, 70 nt, Artificial Sequence
aaaccgagggaucauaggggacugaauccaccauucuucucccaaucccugcaacuccuucuuccccugc

SEQ ID NO: 8 - RNA, 70 nt, Artificial Sequence
ugaacagcuccucgcccuugcucacuggcagagcccuccagcaucgcgagcaggcgcugccuccuccgcc

SEQ ID NO: 9 - DNA, 111 bp, Artificial Sequence
atggacgagctgtacaagctgcagggcggaggaggcagcgcctgctcgcgatgctatagggctctgccagtgagcaagggcgaggagctgttcaccggggtggtgcccatc

SEQ ID NO: 10 - DNA, 111 bp, Artificial Sequence
atggacgagctgtacaagctgcagggcggaggaggcagcgcctgctcgcgatgctaaagggctctgccagtgagcaagggcgaggagctgttcaccggggtggtgcccatc

SEQ ID NO: 11 - DNA, 111 bp, Artificial Sequence
atggacgagctgtacaagctgcagggcggaggaggcagcgcctgctcgcgatgctacagggctctgccagtgagcaagggcgaggagctgttcaccggggtggtgcccatc

SEQ ID NO: 12 - DNA, 111 bp, Artificial Sequence
atggacgagctgtacaagctgcagggcggaggaggcagcgcctgctcgcgatgctagagggctctgccagtgagcaagggcgaggagctgttcaccggggtggtgcccatc

SEQ ID NO: 13 - DNA, 111 bp, Artificial Sequence
atggacgagctgtacaagctgcagggcggaggaggcagcgcctgctcgcgatgcaatagggctctgccagtgagcaagggcgaggagctgttcaccggggtggtgcccatc

SEQ ID NO: 14 - DNA, 111 bp, Artificial Sequence
atggacgagctgtacaagctgcagggcggaggaggcagcgcctgctcgcgatgcaaaagggctctgccagtgagcaagggcgaggagctgttcaccggggtggtgcccatc

SEQ ID NO: 15 - DNA, 111 bp, Artificial Sequence
atggacgagctgtacaagctgcagggcggaggaggcagcgcctgctcgcgatgcaacagggctctgccagtgagcaagggcgaggagctgttcaccggggtggtgcccatc

SEQ ID NO: 16 - DNA, 111 bp, Artificial Sequence
atggacgagctgtacaagctgcagggcggaggaggcagcgcctgctcgcgatgcaagagggctctgccagtgagcaagggcgaggagctgttcaccggggtggtgcccatc

SEQ ID NO: 17 - DNA, 111 bp, Artificial Sequence
atggacgagctgtacaagctgcagggcggaggaggcagcgcctgctcgcgatgccatagggctctgccagtgagcaagggcgaggagctgttcaccggggtggtgcccatc

SEQ ID NO: 18 - DNA, 111 bp, Artificial Sequence
atggacgagctgtacaagctgcagggcggaggaggcagcgcctgctcgcgatgccaaagggctctgccagtgagcaagggcgaggagctgttcaccggggtggtgcccatc

SEQ ID NO: 19 - DNA, 111 bp, Artificial Sequence
atggacgagctgtacaagctgcagggcggaggaggcagcgcctgctcgcgatgccacagggctctgccagtgagcaagggcgaggagctgttcaccggggtggtgcccatc

SEQ ID NO: 20 - DNA, 111 bp, Artificial Sequence
atggacgagctgtacaagctgcagggcggaggaggcagcgcctgctcgcgatgccagagggctctgccagtgagcaagggcgaggagctgttcaccggggtggtgcccatc

SEQ ID NO: 21 - DNA, 111 bp, Artificial Sequence
atggacgagctgtacaagctgcagggcggaggaggcagcgcctgctcgcgatgcgatagggctctgccagtgagcaagggcgaggagctgttcaccggggtggtgcccatc

SEQ ID NO: 22 - DNA, 111 bp, Artificial Sequence
atggacgagctgtacaagctgcagggcggaggaggcagcgcctgctcgcgatgcgaaagggctctgccagtgagcaagggcgaggagctgttcaccggggtggtgcccatc

SEQ ID NO: 23 - DNA, 111 bp, Artificial Sequence
atggacgagctgtacaagctgcagggcggaggaggcagcgcctgctcgcgatgcgacagggctctgccagtgagcaagggcgaggagctgttcaccggggtggtgcccatc

SEQ ID NO: 24 - DNA, 111 bp, Artificial Sequence
atggacgagctgtacaagctgcagggcggaggaggcagcgcctgctcgcgatgcgagagggctctgccagtgagcaagggcgaggagctgttcaccggggtggtgcccatc

SEQ ID NO: 25 - RNA, 91 nt, Artificial Sequence
uagcuguaucgucaaggcacucuugccuacgccaccagcuccaaccaccacaaguuuauauucagucauuuucagcaggccucucucccgc

SEQ ID NO: 26 - RNA, 111 nt, Artificial Sequence
gauucugaauuagcuguaucgucaaggcacucuugccuacgccaccagcuccaacuaccacaaguuuauauucagucauuuucagcaggccucucucccgcaccugggagc

SEQ ID NO: 27 - RNA, 131 nt, Artificial Sequence
uccacaaaaugauucugaauuagcuguaucgucaaggcacucuugccuacgccaccagcuccaacuaccacaaguuuauauucagucauuuucagcaggccucucucccgcaccugggagccgcugagccu

SEQ ID NO: 28 - RNA, 151 nt, Artificial Sequence
aucauauucguccacaaaaugauucugaauuagcuguaucgucaaggcacucuugccuacgccaccagcuccaaccaccacaaguuuauauucagucauuuucagcaggccucucucccgcaccugggagccgcugagccucuggccccgc

SEQ ID NO: 29 - RNA, 171 nt, Artificial Sequence
cuauuguuggaucauauucguccacaaaaugauucugaauuagcuguaucgucaaggcacucuugccuacgccaccagcuccaaccaccacaaguuuauauucagucauuuucagcaggccucucucccgcaccugggagccgcugagccucuggccccgccgccgccuuc

SEQ ID NO: 30 - RNA, 191 nt, Artificial Sequence
uaggaauccucuauuguuggaucauauucguccacaaaaugauucugaauuagcuguaucgucaaggcacucuugccuacgccaccagcuccaaccaccacaaguuuauauucagucauuuucagcaggccucucucccgcaccugggagccgcugagccucuggccccgccgccgccuucagugccugcg

SEQ ID NO: 31 - RNA, 151 nt, Artificial Sequence
gaggcgcagcauccacaggcggaggcgaaagcagcccggacagcugaggccggaagaggguggggccgcgguggccagggagccggcgccgccacgcgcgggugggggggacugggguugcucgcgggcuccgggcgggcggcgggcgccg

SEQ ID NO: 32 - RNA, 151 nt, Artificial Sequence
uccuguagcuaaggccacaaaauuauccacuguuuuuggaacagucuuuccgaagagaccaaagaucacccggcccacaucuucaucuccaauucguaggucaaaauacaccuugacggugacuuugggccccuucuucuucucaucggcc

SEQ ID NO: 33 - RNA, 151 nt, Artificial Sequence
gcccuggaucaugaaguccuugauuacacgauggaauuugcuguuuuuguagccaaauccuuucucuccuguagccaaggccacaaaauuauccacuguuuuuggaacagucuuuccgaagagaccaaagaucacccggccuacaucuuca

SEQ ID NO: 34 - RNA, 72 nt, Artificial Sequence
gcgcaaguuagguuuugucaagaaaggguguaacgcaaccaagucauaguccgccuagaagcauuugcggug

SEQ ID NO: 35 - RNA, 131 nt, Artificial Sequence
gccaugccaaucucaucuuguuuucugcgcaaguuagguuuugucaagaaaggguguaacgcaaccaagucauaguccgccuagaagcauuugcgguggacgauggaggggccggacucgucauacuccug

SEQ ID NO: 36 - RNA, 70 nt, Artificial Sequence
ggacuuccuguaacaacgcaucucauauuuggaaugaccauuaaaaaaacaacaaugugcaaucaaaguc

SEQ ID NO: 37 - RNA, 71 nt, Artificial Sequence
caaggugcggcuccggccccuccccucuucaagggguccacauggcaacugugaggaggggagauucagug

SEQ ID NO: 38 - RNA, 91 nt, Artificial Sequence
uagcuguaucgucaaggcacucgugccgacgccaccagcuccaaccaccacaaggggagagucagucagggucagcaggccucucucccgc

SEQ ID NO: 39 - RNA, 91 nt, Artificial Sequence
uagcuguaucgucaaggcacucuugccgacgccaccagcuccaaccaccacaaguguauagucagucauuuucagcaggccucucucccgc

SEQ ID NO: 40 - RNA, 91 nt, Artificial Sequence
uagcuggaucgucaaggcacucgugccgacgccaccagcuccaaccaccacaaggggagaggcagucagggucagcaggccucucucccgc

SEQ ID NO: 41 - RNA, 111 nt, Artificial Sequence
gauucugaauuagcuguaucgucaaggcacucuugccgacgccaccagcuccaaccaccacaaguguauagucagucauuuucagcaggccucucucccgcaccugggagc

SEQ ID NO: 42 - RNA, 111 nt, Artificial Sequence
gauucugaauuagcuguaucgucaaggcacucgugccgacgccaccagcuccaaccaccacaaguggagagucagucauuuucagcaggccucucucccgcaccugggagc

SEQ ID NO: 43 - RNA, 111 nt, Artificial Sequence
gauucugaauuagcuguaucgucaaggcacucgugccgacgccaccagcuccaaccaccacaaggggagagucagucagggucagcaggccucucucccgcaccugggagc

SEQ ID NO: 44 - RNA, 111 nt, Artificial Sequence
gcuccccggugcgggagagaggccugcugacccugacugccucuccccuuguggugguuggagcugguggcgucggcacgagugccuugacgauccagcuaauucagaauc

SEQ ID NO: 45 - DNA, 71 bp, Artificial Sequence
tctcagtccaatgtatggtccgagcacaagctctaatcaaagtccgcgggtgtagaccggttgccatagga

SEQ ID NO: 46 - RNA, 31 nt, Artificial Sequence
ggaccaccccaaaaaugaaggggacuaaaac

SEQ ID NO: 47 - RNA, 70 nt, Artificial Sequence; identical to SEQ ID NO: 7

SEQ ID NO: 48 - RNA, 14 nt, Artificial Sequence
gcagagccuccagc

SEQ ID NO: 49 - RNA, 21 nt, Artificial Sequence
cucacuggcagagccuccagc

SEQ ID NO: 50 - RNA, 27 nt, Artificial Sequence
cccuugcucacuggcagagccuccagc

SEQ ID NO: 51 - RNA, 33 nt, Artificial Sequence
cucucgcccuugcucacuggcagagccuccagc

SEQ ID NO: 52 - RNA, 38 nt, Artificial Sequence
cucucgcccuugcucacuggcagagccuccagcaucgc

SEQ ID NO: 53 - RNA, 45 nt, Artificial Sequence
ugaacagcucucgcccuugcucacuggcagagccuccagcaucgc

SEQ ID NO: 54 - RNA, 70 nt, Artificial Sequence; identical to SEQ ID NO: 8

SEQ ID NO: 55 - RNA, 70 nt, Artificial Sequence; identical to SEQ ID NO: 7

SEQ ID NO: 56 - RNA, 70 nt, Artificial Sequence; identical to SEQ ID NO: 8

SEQ ID NO: 57 - RNA, 71 nt, Artificial Sequence
ucucaguccaauguaugguccgagcacaagcucuaaucaaaguccgcggguguagaccgguugccauagga

SEQ ID NO: 58 - RNA, 71 nt, Artificial Sequence
acagcuccucgcccuugcucacuggcagagcccuccagcaucgcgagcaggcgcugccuccuccgccgcug

SEQ ID NO: 59 - RNA, 71 nt, Artificial Sequence
acagcuccucgcccuugcucacuggcagagcccucaagcaucgcgagcaggcgcugccuccuccgccgcug

SEQ ID NO: 60 - RNA, 71 nt, Artificial Sequence
acagcuccucgcccuugcucacuggcagagcccucuagcaucgcgagcaggcgcugccuccuccgccgcug

SEQ ID NO: 61 - RNA, 71 nt, Artificial Sequence
acagcuccucgcccuugcucacuggcagagcccucgagcaucgcgagcaggcgcugccuccuccgccgcug

SEQ ID NO: 62 - RNA, 71 nt, Artificial Sequence
acagcuccucgcccuugcucacuggcagagcccugcagcaucgcgagcaggcgcugccuccuccgccgcug

SEQ ID NO: 63 - RNA, 71 nt, Artificial Sequence
acagcuccucgcccuugcucacuggcagagcccuucagcaucgcgagcaggcgcugccuccuccgccgcug

SEQ ID NO: 64 - RNA, 71 nt, Artificial Sequence
acagcuccucgcccuugcucacuggcagagcccuacagcaucgcgagcaggcgcugccuccuccgccgcug

SEQ ID NO: 65 - RNA, 71 nt, Artificial Sequence
acagcuccucgcccuugcucacuggcagagcccuccugcaucgcgagcaggcgcugccuccuccgccgcug

SEQ ID NO: 66 - RNA, 71 nt, Artificial Sequence
acagcuccucgcccuugcucacuggcagagcccugcugcaucgcgagcaggcgcugccuccuccgccgcug

SEQ ID NO: 67 - RNA, 71 nt, Artificial Sequence
acagcuccucgcccuugcucacuggcagagcccuucugcaucgcgagcaggcgcugccuccuccgccgcug

SEQ ID NO: 68 - RNA, 71 nt, Artificial Sequence
acagcuccucgcccuugcucacuggcagagcccuacugcaucgcgagcaggcgcugccuccuccgccgcug

SEQ ID NO: 69 - RNA, 71 nt, Artificial Sequence
acagcuccucgcccuugcucacuggcagagcccucccgcaucgcgagcaggcgcugccuccuccgccgcug

SEQ ID NO: 70 - RNA, 71 nt, Artificial Sequence
acagcuccucgcccuugcucacuggcagagcccugccgcaucgcgagcaggcgcugccuccuccgccgcug

SEQ ID NO: 71 - RNA, 71 nt, Artificial Sequence
acagcuccucgcccuugcucacuggcagagcccuuccgcaucgcgagcaggcgcugccuccuccgccgcug

SEQ ID NO: 72 - RNA, 71 nt, Artificial Sequence
acagcuccucgcccuugcucacuggcagagcccuaccgcaucgcgagcaggcgcugccuccuccgccgcug

SEQ ID NO: 73 - RNA, 71 nt, Artificial Sequence
acagcuccucgcccuugcucacuggcagagcccuccggcaucgcgagcaggcgcugccuccuccgccgcug

SEQ ID NO: 74 - RNA, 71 nt, Artificial Sequence; identical to SEQ ID NO: 66

SEQ ID NO: 75 - RNA, 71 nt, Artificial Sequence
acagcuccucgcccuugcucacuggcagagcccuucggcaucgcgagcaggcgcugccuccuccgccgcug

SEQ ID NO: 76 - RNA, 71 nt, Artificial Sequence
acagcuccucgcccuugcucacuggcagagcccuacggcaucgcgagcaggcgcugccuccuccgccgcug

SEQ ID NO: 77 - RNA, 31 nt, Artificial Sequence
acuggcagagcccuccagcaucgcgagcagg

SEQ ID NO: 78 - RNA, 51 nt, Artificial Sequence
gcccuugcucacuggcagagcccuccagcaucgcgagcaggcgcugccucc

SEQ ID NO: 79 - RNA, 71 nt, Artificial Sequence; identical to SEQ ID NO: 58

SEQ ID NO: 80 - RNA, 91 nt, Artificial Sequence
accccggugaacagcuccucgcccuugcucacuggcagagcccuccagcaucgcgagcaggcgcugccuccuccgccgcugccuccuccgc

SEQ ID NO: 81 - RNA, 131 nt, Artificial Sequence
gcucgaccaggaugggcaccaccccggugaacagcuccucgcccuugcucacuggcagagcccuccagcaucgcgagcaggcgcugccuccuccgccgcugccuccuccgccgcugccuccuccgcccugc

SEQ ID NO: 82 - RNA, 151 nt, Artificial Sequence
ucgccguccagcucgaccaggaugggcaccaccccggugaacagcuccucgcccuugcucacuggcagagcccuccagcaucgcgagcaggcgcugccuccuccgccgcugccuccuccgccgcugccuccuccgcccugcagcuuguaca

SEQ ID NO: 83 - RNA, 171 nt, Artificial Sequence
gccguuuacgucgccguccagcucgaccaggaugggcaccaccccggugaacagcuccucgcccuugcucacuggcagagcccuccagcaucgcgagcaggcgcugccuccuccgccgcugccuccuccgccgcugccuccuccgcccugcagcuuguacagcucguccau

SEQ ID NO: 84 - RNA, 191 nt, Artificial Sequence
ugaacuuguggccguuuacgucgccguccagcucgaccaggaugggcaccaccccggugaacagcuccucgcccuugcucacuggcagagcccuccagcaucgcgagcaggcgcugccuccuccgccgcugccuccuccgccgcugccuccuccgcccugcagcuuguacagcucguccaugccgccggug

SEQ ID NO: 85 - RNA, 211 nt, Artificial Sequence
ccggacacgcugaacuuguggccguuuacgucgccguccagcucgaccaggaugggcaccaccccggugaacagcuccucgcccuugcucacuggcagagcccuccagcaucgcgagcaggcgcugccuccuccgccgcugccuccuccgccgcugccuccuccgcccugcagcuuguacagcucguccaugccgccgguggaguggcggc

SEQ ID NO: 86 - RNA, 31 nt, Artificial Sequence
gcgaccggggaucuccacagauucuuccggc

SEQ ID NO: 87 - RNA, 51 nt, Artificial Sequence
gcucacgguggcgaccggggaucuccacagauucuuccggcguguauaccu

SEQ ID NO: 88 - RNA, 71 nt, Artificial Sequence
ccucgcccuugcucacgguggcgaccggggaucuccacagauucuuccggcguguauaccuucugcugccu

SEQ ID NO: 89 - RNA, 91 nt, Artificial Sequence
gugaacagcuccucgcccuugcucacgguggcgaccggggaucuccacagauucuuccggcguguauaccuucugcugccuccuccgccgc

SEQ ID NO: 90 - RNA, 111 nt, Artificial Sequence
caccaccccggugaacagcuccucgcccuugcucacgguggcgaccggggaucuccacagauucuuccggcguguauaccuucugcugccuccuccgccgcugccuccucc

SEQ ID NO: 91 - RNA, 131 nt, Artificial Sequence
ccaggaugggcaccaccccggugaacagcuccucgcccuugcucacgguggcgaccggggaucuccacagauucuuccggcguguauaccuucugcugccuccuccgccgcugccuccuccgccgcugccu

SEQ ID NO: 92 - RNA, 151 nt, Artificial Sequence
uccagcucgaccaggaugggcaccaccccggugaacagcuccucgcccuugcucacgguggcgaccggggaucuccacagauucuuccggcguguauaccuucugcugccuccuccgccgcugccuccuccgccgcugccuccuccgcccu

SEQ ID NO: 93 - RNA, 171 nt, Artificial Sequence
cggcgacguauccagcucgaccaggaugggcaccaccccggugaacagcuccucgcccuugcucacgguggcgaccggggaucuccacagauucuuccggcguguauaccuucugcugccuccuccgccgcugccuccuccgccgcugccuccuccgcccugcagcuugua

SEQ ID NO: 94 - RNA, 191 nt, Artificial Sequence
uguggccguuuacgucgccguccagcucgaccaggaugggcaccaccccggugaacagcuccucgcccuugcucacgguggcgaccggggaucuccacagauucuuccggcguguauaccuucugcugccuccuccgccgcugccuccuccgccgcugccuccuccgcccugcagcuuguacagcucgucc

SEQ ID NO: 95 - RNA, 211 nt, Artificial Sequence
acgcugaacuuguggccguuuacgucgccguccagcucgaccaggaugggcaccaccccggugaacagcuccucgcccuugcucacgguggcgaccggggaucuccacagauucuuccggcguguauaccuucugcugccuccuccgccgcugccuccuccgccgcugccuccuccgcccugcagcuuguacagcucguccaugccgccgg

SEQ ID NO: 96 - RNA, 71 nt, Artificial Sequence
cagcaucgcgagcaggcgcugccuccuccgccgcugccuccuccgccgcugccuccuccgcccugcagcuu

SEQ ID NO: 97 - RNA, 71 nt, Artificial Sequence
cccuccagcaucgcgagcaggcgcugccuccuccgccgcugccuccuccgccgcugccuccuccgcccugc

SEQ ID NO: 98 - RNA, 71 nt, Artificial Sequence
cagagcccuccagcaucgcgagcaggcgcugccuccuccgccgcugccuccuccgccgcugccuccuccgc

SEQ ID NO: 99 - RNA, 72 nt, Artificial Sequence
acuggcagagcccucccagcaucgcgagcaggcgcugccuccuccgccgcugccuccuccgccgcugccucc

SEQ ID NO: 100 - RNA, 71 nt, Artificial Sequence
ugcucacuggcagagcccuccagcaucgcgagcaggcgcugccuccuccgccgcugccuccuccgccgcug

SEQ ID NO: 101 - RNA, 71 nt, Artificial Sequence
gcccuugcucacuggcagagcccuccagcaucgcgagcaggcgcugccuccuccgccgcugccuccuccgc

SEQ ID NO: 102 - RNA, 71 nt, Artificial Sequence
uccucgcccuugcucacuggcagagcccuccagcaucgcgagcaggcgcugccuccuccgccgcugccucc

SEQ ID NO: 103 - RNA, 71 nt, Artificial Sequence
ggugaacagcuccucgcccuugcucacuggcagagcccuccagcaucgcgagcaggcgcugccuccuccgc

SEQ ID NO: 104 - RNA, 71 nt, Artificial Sequence
accccggugaacagcuccucgcccuugcucacuggcagagcccuccagcaucgcgagcaggcgcugccucc

SEQ ID NO: 105 - RNA, 71 nt, Artificial Sequence
gcaccaccccggugaacagcuccucgcccuugcucacuggcagagcccuccagcaucgcgagcaggcgcug

SEQ ID NO: 106 - RNA, 71 nt, Artificial Sequence
gaugggcaccaccccggugaacagcuccucgcccuugcucacuggcagagcccuccagcaucgcgagcagg

SEQ ID NO: 107 - RNA, 71 nt, Artificial Sequence
accaggaugggcaccaccccggugaacagcuccucgcccuugcucacuggcagagcccuccagcaucgcga

SEQ ID NO: 108 - RNA, 71 nt, Artificial Sequence
gcucgaccaggaugggcaccaccccggugaacagcuccucgcccuugcucacuggcagagcccuccagcau

SEQ ID NO: 109 - RNA, 71 nt, Artificial Sequence
guccagcucgaccaggaugggcaccaccccggugaacagcuccucgcccuugcucacuggcagagcccucc

SEQ ID NO: 110 - RNA, 71 nt, Artificial Sequence
cacagauucuuccggcguguauaccuucugcugccuccuccgccgcugccuccuccgccgcugccuccucc

SEQ ID NO: 111 - RNA, 71 nt, Artificial Sequence
aucuccacagauucuuccggcguguauaccuucugcugccuccuccgccgcugccuccuccgccgcugccu

SEQ ID NO: 112 - RNA, 71 nt, Artificial Sequence
cggggaucuccacagauucuuccggcguguauaccuucugcugccuccuccgccgcugccuccuccgccgc

SEQ ID NO: 113 - RNA, 71 nt, Artificial Sequence
gcgaccggggaucuccacagauucuuccggcguguauaccuucugcugccuccuccgccgcugccuccucc

SEQ ID NO: 114 - RNA, 71 nt, Artificial Sequence
cgguggcgaccggggaucuccacagauucuuccggcguguauaccuucugcugccuccuccgccgcugccu

SEQ ID NO: 115 - RNA, 71 nt, Artificial Sequence
gcucacgguggcgaccggggaucuccacagauucuuccggcguguauaccuucugcugccuccuccgccgc

SEQ ID NO: 116 - RNA, 71 nt, Artificial Sequence
cccuugcucacgguggcgaccggggaucuccacagauucuuccggcguguauaccuucugcugccuccucc

SEQ ID NO: 117 - RNA, 71 nt, Artificial Sequence
cagcuccucgcccuugcucacgguggcgaccggggaucuccacagauucuuccggcguguauaccuucugc

SEQ ID NO: 118 - RNA, 71 nt, Artificial Sequence
gugaacagcuccucgcccuugcucacgguggcgaccggggaucuccacagauucuuccggcguguauaccu

SEQ ID NO: 119 - RNA, 71 nt, Artificial Sequence
ccccggugaacagcuccucgcccuugcucacgguggcgaccggggaucuccacagauucuuccggcgugua

SEQ ID NO: 120 - RNA, 71 nt, Artificial Sequence
caccaccccggugaacagcuccucgcccuugcucacgguggcgaccggggaucuccacagauucuuccggc

SEQ ID NO: 121 - RNA, 71 nt, Artificial Sequence
augggcaccaccccggugaacagcuccucgcccuugcucacgguggcgaccggggaucuccacagauucuu

SEQ ID NO: 122 - RNA, 71 nt, Artificial Sequence
ccaggaugggcaccaccccggugaacagcuccucgcccuugcucacgguggcgaccggggaucuccacaga

SEQ ID NO: 123 - RNA, 71 nt, Artificial Sequence
cucgaccaggaugggcaccaccccggugaacagcuccucgcccuugcucacgguggcgaccggggaucucc

SEQ ID NO: 124 - RNA, 111 nt, Artificial Sequence
gaugggcaccaccccggugaacagcuccucgcccuugcucacuggcagagcccuccagcaucgcgagcaggcgcugccuccuccgcccugcagcuuguacagcucguccau

SEQ ID NO: 125 - RNA, 111 nt, Artificial Sequence
gaugggcaccaccccggugaacagcuccucgcccuugcucacuggcagagcccugcagcaucgcgagcaggcgcugccuccuccgcccugcagcuuguacagcucguccau

SEQ ID NO: 126 - RNA, 111 nt, Artificial Sequence
gaugggcaccaccccggugaacagcuccucgcccuugcucacuggcagagcccuucagcaucgcgagcaggcgcugccuccuccgcccugcagcuuguacagcucguccau

SEQ ID NO: 127 - RNA, 111 nt, Artificial Sequence
gaugggcaccaccccggugaacagcuccucgcccuugcucacuggcagagcccuacagcaucgcgagcaggcgcugccuccuccgcccugcagcuuguacagcucguccau

SEQ ID NO: 128 - RNA, 111 nt, Artificial Sequence
gaugggcaccaccccggugaacagcuccucgcccuugcucacuggcagagcccuccggcaucgcgagcaggcgcugccuccuccgcccugcagcuuguacagcucguccau

SEQ ID NO: 129 - RNA, 111 nt, Artificial Sequence
gaugggcaccaccccggugaacagcuccucgcccuugcucacuggcagagcccugcggcaucgcgagcaggcgcugccuccuccgcccugcagcuuguacagcucguccau

SEQ ID NO: 130 - RNA, 111 nt, Artificial Sequence
gaugggcaccaccccggugaacagcuccucgcccuugcucacuggcagagcccuucggcaucgcgagcaggcgcugccuccuccgcccugcagcuuguacagcucguccau

SEQ ID NO: 131 - RNA, 111 nt, Artificial Sequence
gaugggcaccaccccggugaacagcuccucgcccuugcucacuggcagagcccuacggcaucgcgagcaggcgcugccuccuccgcccugcagcuuguacagcucguccau

SEQ ID NO: 132 - RNA, 111 nt, Artificial Sequence
gaugggcaccaccccggugaacagcuccucgcccuugcucacuggcagagcccuccugcaucgcgagcaggcgcugccuccuccgcccugcagcuuguacagcucguccau

SEQ ID NO: 133 - RNA, 111 nt, Artificial Sequence
gaugggcaccaccccggugaacagcuccucgcccuugcucacuggcagagcccugcugcaucgcgagcaggcgcugccuccuccgcccugcagcuuguacagcucguccau

SEQ ID NO: 134 - RNA, 111 nt, Artificial Sequence
gaugggcaccaccccggugaacagcuccucgcccuugcucacuggcagagcccuacugcaucgcgagcaggcgcugccuccuccgcccugcagcuuguacagcucguccau

SEQ ID NO: 135 - RNA, 111 nt, Artificial Sequence
gaugggcaccaccccggugaacagcuccucgcccuugcucacuggcagagcccuucugcaucgcgagcaggcgcugccuccuccgcccugcagcuuguacagcucguccau

SEQ ID NO: 136 - RNA, 111 nt, Artificial Sequence
gaugggcaccaccccggugaacagcuccucgcccuugcucacuggcagagcccucccgcaucgcgagcaggcgcugccuccuccgcccugcagcuuguacagcucguccau

SEQ ID NO: 137 - RNA, 111 nt, Artificial Sequence
gaugggcaccaccccggugaacagcuccucgcccuugcucacuggcagagcccugccgcaucgcgagcaggcgcugccuccuccgcccugcagcuuguacagcucguccau

SEQ ID NO: 138 - RNA, 111 nt, Artificial Sequence
gaugggcaccaccccggugaacagcuccucgcccuugcucacuggcagagcccuuccgcaucgcgagcaggcgcugccuccuccgcccugcagcuuguacagcucguccau

SEQ ID NO: 139 - RNA, 111 nt, Artificial Sequence
gaugggcaccaccccggugaacagcuccucgcccuugcucacuggcagagcccuaccgcaucgcgagcaggcgcugccuccuccgcccugcagcuuguacagcucguccau

SEQ ID NO: 140 - RNA, 111 nt, Artificial Sequence
uaccgcuacagccacgcugauuucagcuauaccugcccgguauaaagggacguucacaccgcgauguucucugcuggggaauugcgcgauauucaggauuaaaagaagugc

SEQ ID NO: 141 - RNA, 151 nt, Artificial Sequence
acuacaguugcuccgauauuuaggcuacgucaauaggcacuaacuuauuggcgcuggugaacggacuuccucucgaguaccagaagaugacuacaaaacuccuuuccauugcgaguaucggagucuggcucaguuuggccagggaggcacu

SEQ ID NO: 142 - RNA, 51 nt, Artificial Sequence
cggaagaggguggggccgcgguggccagggagccggcgccgccacgcgcgg

SEQ ID NO: 143 - RNA, 71 nt, Artificial Sequence
cagcugaggccggaagaggguggggccgcgguggccagggagccggcgccgccacgcgcggguggggggga

SEQ ID NO: 144 - RNA, 111 nt, Artificial Sequence
ggaggcgaaagcagcccggacagcugaggccggaagaggguggggccgcgguggccagggagccggcgccgccacgcgcgggugggggggacugggguugcucgcgggcuc

SEQ ID NO: 145 - RNA, 151 nt, Artificial Sequence; identical to SEQ ID NO: 31

SEQ ID NO: 146 - RNA, 51 nt, Artificial Sequence
ucuugccuacgccaccagcuccaaccaccacaaguuuauauucagucauuu

SEQ ID NO: 147 - RNA, 111 nt, Artificial Sequence
gauucugaauuagcuguaucgucaaggcacucuugccuacgccaccagcuccaaccaccacaaguuuauauucagucauuuucagcaggccucucucccgcaccugggagc

SEQ ID NO: 148 - RNA, 151 nt, Artificial Sequence; identical to SEQ ID NO: 28

SEQ ID NO: 149 - RNA, 51 nt, Artificial Sequence
ucggcaugguaugaaguacuucguccaggagcuggagggcccgguguaagu

SEQ ID NO: 150 - RNA, 71 nt, Artificial Sequence
gggucugcaaucggcaugguaugaaguacuucguccaggagcuggagggcccgguguaagugaauuucaau

SEQ ID NO: 151 - RNA, 111 nt, Artificial Sequence
gaccucagucuaaagguugugggucugcaaucggcaugguaugaaguacuucguccaggagcuggagggcccgguguaagugaauuucaauccagcaagguguuucuuuga

SEQ ID NO: 152 - RNA, 151 nt, Artificial Sequence
uaagggccccaacgguaaaagaccucagucuaaagguugugggucugcaaucggcaugguaugaaguacuucguccaggagcuggagggcccgguguaagugaauuucaauccagcaagguguuucuuugaugcucugucuuggguaaucc

SEQ ID NO: 153 - RNA, 51 nt, Artificial Sequence
ugggggguucggcugccgacaucagcaauugcucugccaccaucucagccc

SEQ ID NO: 154 - RNA, 71 nt, Artificial Sequence
agcagggccgugggggguucggcugccgacaucagcaauugcucugccaccaucucagcccauccuccgaa

SEQ ID NO: 155 - RNA, 111 nt, Artificial Sequence
aguagaaggccaagagccacagcagggccgugggggguucggcugccgacaucagcaauugcucugccaccaucucagcccauccuccgaagugaaugaacaggaaccagc

SEQ ID NO: 156 - RNA, 151 nt, Artificial Sequence
ccucccaucacgggggccguaguagaaggccaagagccacagcagggccgugggggguucggcugccgacaucagcaauugcucugccaccaucucagcccauccuccgaagugaaugaacaggaaccagcucucaaagggaccuccgcag

SEQ ID NO: 157 - DNA, 151 bp, Artificial Sequence
gccaaacaccacatgcttgccatctagccaggctgtcttgactgtcgtgatgaagaactgggagccgttggtgtccttgcctgcgttggccatgctcacccagccaggcccgtagtgcttcagtttgaagttctcatcggggaagcgctca

SEQ ID NO: 158 - DNA, 151 bp, Artificial Sequence
gggagtgggtccgctccaccagatgccagcaccggggccagtgcagctcagagccctgtggcggactacagggcccgcacagacggtcactcaaagaaagatgtccctgtgccctactccttggcgatggcaaagggcttctccacctcga

SEQ ID NO: 159 - DNA, 151 bp, Artificial Sequence
tgcattttgtaaaatagatactagcagattgtcccaagatgtgtacagctcattctcacagcccagcgagggcacctactccacaaatgcgtggccacaggtcatcacctgtcctgtggccctggcgagcctgatccctcacgccgggcac

SEQ ID NO: 160 - DNA, 151 bp, Artificial Sequence
gctcattctcacagcccagcgagggcacttactccacaaatgcgtggccacaggtcatcacctgtcctgtggccccggcgagcctgatccctcacgccgggcacccacacggcctgcgtgccttctagacttgagttcgcagctctttaag

SEQ ID NO: 161 - DNA, 151 bp, Artificial Sequence
tcggccgggccctgggggcggtgggcgctggccaggacgcccaccgtgtggttgctgtccaggacggtcccggcccgcgacacttcggcccagagctgctcctcatccagcagcgccagcagccccatggccgtgagcaccggcttgcgca

SEQ ID NO: 162 - RNA, 111 nt, Artificial Sequence
ugaccagucuuaagaucuuucuugaccugcaccauaagaacuucuccaaagguaccaaaauacucuuucagguccuguucgguuguuuuccaugggagacccaacacuauu

SEQ ID NO: 163 - RNA, 111 nt, Artificial Sequence
gaugggcaccaccccggugaacagcuccucgcccuugcucacuggcagagcccucgagcaucgcgagcaggcgcugccuccuccgcccugcagcuuguacagcucguccau

SEQ ID NO: 164 - RNA, 111 nt, Artificial Sequence
gaugggcaccaccccggugaacagcuccucgcccuugcucacuggcagagcccuggagcaucgcgagcaggcgcugccuccuccgcccugcagcuuguacagcucguccau

SEQ ID NO: 165 - RNA, 111 nt, Artificial Sequence
gaugggcaccaccccggugaacagcuccucgcccuugcucacuggcagagcccuugagcaucgcgagcaggcgcugccuccuccgcccugcagcuuguacagcucguccau

SEQ ID NO: 166 - RNA, 111 nt, Artificial Sequence
gaugggcaccaccccggugaacagcuccucgcccuugcucacuggcagagcccuagagcaucgcgagcaggcgcugccuccuccgcccugcagcuuguacagcucguccau

SEQ ID NO: 167 - RNA, 111 nt, Artificial Sequence
gaugggcaccaccccggugaacagcuccucgcccuugcucacuggcagagcccucgggcaucgcgagcaggcgcugccuccuccgcccugcagcuuguacagcucguccau

SEQ ID NO: 168 - RNA, 111 nt, Artificial Sequence
gaugggcaccaccccggugaacagcuccucgcccuugcucacuggcagagcccuggggcaucgcgagcaggcgcugccuccuccgcccugcagcuuguacagcucguccau

SEQ ID NO: 169 - RNA, 111 nt, Artificial Sequence
gaugggcaccaccccggugaacagcuccucgcccuugcucacuggcagagcccuugggcaucgcgagcaggcgcugccuccuccgcccugcagcuuguacagcucguccau

SEQ ID NO: 170 - RNA, 111 nt, Artificial Sequence
gaugggcaccaccccggugaacagcuccucgcccuugcucacuggcagagcccuagggcaucgcgagcaggcgcugccuccuccgcccugcagcuuguacagcucguccau

SEQ ID NO: 171 - RNA, 111 nt, Artificial Sequence
gaugggcaccaccccggugaacagcuccucgcccuugcucacuggcagagcccucgugcaucgcgagcaggcgcugccuccuccgcccugcagcuuguacagcucguccau

SEQ ID NO: 172 - RNA, 111 nt, Artificial Sequence
gaugggcaccaccccggugaacagcuccucgcccuugcucacuggcagagcccuggugcaucgcgagcaggcgcugccuccuccgcccugcagcuuguacagcucguccau

SEQ ID NO: 173 - RNA, 111 nt, Artificial Sequence
gaugggcaccaccccggugaacagcuccucgcccuugcucacuggcagagcccuagugcaucgcgagcaggcgcugccuccuccgcccugcagcuuguacagcucguccau

SEQ ID NO: 174 - RNA, 111 nt, Artificial Sequence
gaugggcaccaccccggugaacagcuccucgcccuugcucacuggcagagcccuugugcaucgcgagcaggcgcugccuccuccgcccugcagcuuguacagcucguccau

SEQ ID NO: 175 - RNA, 111 nt, Artificial Sequence
gaugggcaccaccccggugaacagcuccucgcccuugcucacuggcagagcccucgcgcaucgcgagcaggcgcugccuccuccgcccugcagcuuguacagcucguccau

SEQ ID NO: 176 - RNA, 111 nt, Artificial Sequence
gaugggcaccaccccggugaacagcuccucgcccuugcucacuggcagagcccuggcgcaucgcgagcaggcgcugccuccuccgcccugcagcuuguacagcucguccau

SEQ ID NO: 177 - RNA, 111 nt, Artificial Sequence
gaugggcaccaccccggugaacagcuccucgcccuugcucacuggcagagcccuugcgcaucgcgagcaggcgcugccuccuccgcccugcagcuuguacagcucguccau

SEQ ID NO: 178 - RNA, 111 nt, Artificial Sequence
gaugggcaccaccccggugaacagcuccucgcccuugcucacuggcagagcccuagcgcaucgcgagcaggcgcugccuccuccgcccugcagcuuguacagcucguccau

SEQ ID NO: 179 - RNA, 111 nt, Artificial Sequence; identical to SEQ ID NO: 163

SEQ ID NO: 180 - RNA, 111 nt, Artificial Sequence; identical to SEQ ID NO: 164

SEQ ID NO: 181 - RNA, 111 nt, Artificial Sequence; identical to SEQ ID NO: 165

SEQ ID NO: 182 - RNA, 111 nt, Artificial Sequence; identical to SEQ ID NO: 166

SEQ ID NO: 183 - RNA, 111 nt, Artificial Sequence; identical to SEQ ID NO: 171

SEQ ID NO: 184 - RNA, 111 nt, Artificial Sequence; identical to SEQ ID NO: 167

SEQ ID NO: 185 - RNA, 111 nt, Artificial Sequence; identical to SEQ ID NO: 175

SEQ ID NO: 186 - RNA, 111 nt, Artificial Sequence; identical to SEQ ID NO: 171

SEQ ID NO: 187 - RNA, 111 nt, Artificial Sequence; identical to SEQ ID NO: 172

SEQ ID NO: 188 - RNA, 111 nt, Artificial Sequence; identical to SEQ ID NO: 174

SEQ ID NO: 189 - RNA, 111 nt, Artificial Sequence; identical to SEQ ID NO: 173

SEQ ID NO: 190 - RNA, 111 nt, Artificial Sequence; identical to SEQ ID NO: 163

SEQ ID NO: 191 - RNA, 111 nt, Artificial Sequence; identical to SEQ ID NO: 175

SEQ ID NO: 192 - RNA, 111 nt, Artificial Sequence; identical to SEQ ID NO: 167

SEQ ID NO: 193 - RNA, 111 nt, Artificial Sequence; identical to SEQ ID NO: 42

SEQ ID NO: 194 - RNA, 111 nt, Artificial Sequence
gauucugaauuagcuggaucgucaaggcacucgggccgacgccaccagcuccaaccaccacaaguggagagucagucauuuucagcaggccucucucccgcaccggggagc

SEQ ID NO: 195 - RNA, 111 nt, Artificial Sequence
gggagcagccucuggcauucugggagcuucaucuggaccugggucuucagugaaccauuguucaauaucguccggggacagcaucaaaucauccauugcuugggacggcaa

SEQ ID NO: 196 - RNA, 111 nt, Artificial Sequence
gggagcagccucuggcauucugggagcuucaucuggaccugggucuucagugaaccauuguucaagaucguccggggacagcaucaaaucauccauugcuugggacggcaa

SEQ ID NO: 197 - RNA, 111 nt, Artificial Sequence
gggagcagccucuggcagucggggagcuucaucuggaccugggucuucagugaaccauuguucaagaucguccggggacagcaucaaaucauccagugcuugggacggcaa

SEQ ID NO: 198 - RNA, 111 nt, Artificial Sequence
cauauuacagaauaccuugauagcauccaauuugcauccuugguuagggucaacccaguauucuccacucuugaguucaggauggcagaauuucaggucucugcaguuucu

SEQ ID NO: 199 - RNA, 111 nt, Artificial Sequence
gugaagauaagccaguccucuaguaacagaaugagcaagacggcaagagcuuacccagucacuuguguggagacuuaaauacuugcauaaagauccauugggauaguacuc

SEQ ID NO: 200 - RNA, 111 nt, Artificial Sequence
gugaacgucaaacugucggaccaauauggcagaaucuucucucaucucaacuuuccauauccguaucauggaaucauagcauccuguaacuacuagcucucuuacagcugg

SEQ ID NO: 201 - RNA, 111 nt, Artificial Sequence
gccaaugaucucgugaguuaucucagcagugugagccaucagggugaugacaucccaggcgaucguguggccuccaggagcccagagcaggaaguugaggagaaggugccu

SEQ ID NO: 202 - RNA, 111 nt, Artificial Sequence
caagacggugaaccacuccauggucuucuugucggcuuucugcacuguguacccccagagcuccguguugccgacauccugggguggcuuccacuccagagccacauuaag

SEQ ID NO: 203 - RNA, 111 nt, Artificial Sequence
aggauucucuuuugaaguauugcucccccaguggauuggguggcuccauucacuccaaugcugagcacuuccacagaguggguuaaagcggcuccgaacacgaaacgugua

SEQ ID NO: 204 - RNA, 111 nt, Artificial Sequence
gacgcccaccgugugguugcuguccaggacggucccggccugcgacacuucggcccagagcugcuccucauccagcagcgccagcagccccauggccgugagcaccggcuu

SEQ ID NO: 205 - RNA, 111 nt, Artificial Sequence
gacgcccaccgugugguugcuguccaggacggucccggccugcgacacuucggcccagagcugcuccucaucugcggggcgggggggggccgucgccgcguggggucguug

SEQ ID NO: 206 - DNA, 31 bp, Artificial Sequence
tataactagtatggtgagcaagggcgaggag

SEQ ID NO: 207 - DNA, 41 bp, Artificial Sequence
tatacgtctcatctacagattcttccggcgtgtataccttc

SEQ ID NO: 208 - DNA, 53 bp, Artificial Sequence
tatacgtctcatagagatccccggtcgccaccgtgagcaagggcgaggagctg

SEQ ID NO: 209 - DNA, 36 bp, Artificial Sequence
tataggcgcgccttacttgtacagctcgtccatgcc

SEQ ID NO: 210 - DNA, 94 bp, Artificial Sequence
tatacgtctcaaggcgctgcctcctccgccgctgcctcctccgccgctgcctcctccgccctgcagcttgtacagctcgtccatgccgccggtg

SEQ ID NO: 211 - DNA, 62 bp, Artificial Sequence
tatacgtctcagcctgctcgcgatgctagagggctctgccagtgagcaagggcgaggagctg

SEQ ID NO: 212 - DNA, 70 bp, Artificial Sequence
tataactagtatggtggattacaaggatgacgacgataagatgaaagtgacgaaggtaggaggcatttcg

SEQ ID NO: 213 - DNA, 60 bp, Artificial Sequence
atatggcgcgccgttttcagactttttctcttccattttgtattcaaacataatcttcac

SEQ ID NO: 214 - DNA, 69 bp, Artificial Sequence
tataggcgcgccaggcggaggaggcagcggcggaggaggcagcctcctcctctcaaggtccccagaagc

SEQ ID NO: 215 - DNA, 64 bp, Artificial Sequence
tatacctgcaggctacaccttgcgttttttcttgggtactgggcagagataaaagttcttttcc

SEQ ID NO: 216 - DNA, 24 bp, Artificial Sequence
cactccaccggcggcatggacgag

SEQ ID NO: 217 - DNA, 28 bp, Artificial Sequence
cacgctgaacttgtggccgtttacgtcg

SEQ ID NO: 218 - DNA, 40 bp, Artificial Sequence
tataactagtatgaatccgcggcaggggtattccctcagc

SEQ ID NO: 219 - DNA, 73 bp, Artificial Sequence
tataggcgcgccctacttatcgtcgtcatccttgtaatctactgggcagagataaaagttcttttcctcctgg

SEQ ID NO: 220 - DNA, 42 bp, Artificial Sequence
tataactagtatggatatagaagatgaagaaaacatgagttc

SEQ ID NO: 221 - DNA, 67 bp, Artificial Sequence
tataggcgcgccctacttatcgtcgtcatccttgtaatcgggcgtgagtgagaactggtcctgctcg

SEQ ID NO: 222 - DNA, 37 bp, Artificial Sequence
tataactagtatggccgagatcaaggagaaaatctgc

SEQ ID NO: 223 - DNA, 73 bp, Artificial Sequence; identical to SEQ ID NO: 219

SEQ ID NO: 224 - DNA, 19 bp, Artificial Sequence
cgccatttcggactgggag

SEQ ID NO: 225 - DNA, 25 bp, Artificial Sequence
agagacaggtttctccatcaattac

SEQ ID NO: 226 - DNA, 16 bp, Artificial Sequence
gagcccgcgagcaacc

SEQ ID NO: 227 - DNA, 20 bp, Artificial Sequence
gcagcaggaagaagacggac

SEQ ID NO: 228 - DNA, 23 bp, Artificial Sequence
agaagcagttgaagaccagactc

SEQ ID NO: 229 - DNA, 20 bp, Artificial Sequence
ggccttcacctggaccatag

SEQ ID NO: 230 - DNA, 22 bp, Artificial Sequence
agagaagcagttgaagaccaga

SEQ ID NO: 231 - DNA, 20 bp, Artificial Sequence
cggccttcacctggaccata

SEQ ID NO: 232 - DNA, 23 bp, Artificial Sequence
cagagaagcagttgaagaccaga

SEQ ID NO: 233 - DNA, 20 bp, Artificial Sequence
cggccttcacctggaccata

SEQ ID NO: 234 - DNA, 20 bp, Artificial Sequence
tttgtgaaaggctggggacc

SEQ ID NO: 235 - DNA, 25 bp, Artificial Sequence
acaggattgtattttgtagtccacc

SEQ ID NO: 236 - DNA, 23 bp, Artificial Sequence
aggatgagttttgtgaaaggctg

SEQ ID NO: 237 - DNA, 24 bp, Artificial Sequence
attttgtagtccaccatcctgata

SEQ ID NO: 238 - DNA, 22 bp, Artificial Sequence
gatgagttttgtgaaaggctgg

SEQ ID NO: 239 - DNA, 25 bp, Artificial Sequence
attttgtagtccaccatcctgataa

SEQ ID NO: 240 - DNA, 20 bp, Artificial Sequence
cgaagagaacgagaccgcat

SEQ ID NO: 241 - DNA, 19 bp, Artificial Sequence
gaagatggtgcacaccggg

SEQ ID NO: 242 - DNA, 22 bp, Artificial Sequence
gacagatgcttcatcagcagtg

SEQ ID NO: 243 - DNA, 21 bp, Artificial Sequence
cgaacaaagccaaaccccttt

SEQ ID NO: 244 - DNA, 25 bp, Artificial Sequence
tctgttaatggacaaatagaaagcc

SEQ ID NO: 245 - DNA, 23 bp, Artificial Sequence
ggaacattcaaaggattggcact

SEQ ID NO: 246 - DNA, 20 bp, Artificial Sequence
agtcactgcagatggacgca

SEQ ID NO: 247 - DNA, 22 bp, Artificial Sequence
atctcgatgggaaattgcaggt

SEQ ID NO: 248 - DNA, 25 bp, Artificial Sequence
tcagagttttacctcatccttcttt

SEQ ID NO: 249 - DNA, 25 bp, Artificial Sequence
cctgaatacatatgatgaccttcag

SEQ ID NO: 250 - DNA, 20 bp, Artificial Sequence
agggcacagacacagacctc

SEQ ID NO: 251 - DNA, 21 bp, Artificial Sequence
agggctttcaatgccaagacg

SEQ ID NO: 252 - DNA, 19 bp, Artificial Sequence
tgacaagccaagtcctccc

SEQ ID NO: 253 - DNA, 21 bp, Artificial Sequence
attgccaatgatgagctctgg

SEQ ID NO: 254 - DNA, 25 bp, Artificial Sequence
ttatagacataagttctccttgcct

SEQ ID NO: 255 - DNA, 20 bp, Artificial Sequence
tcaatcccatggagccaaca

SEQ ID NO: 256 - DNA, 50 bp, Artificial Sequence
tacacgacgctcttccgatcttaagtagaggccgccactccaccggcggc

SEQ ID NO: 257 - DNA, 51 bp, Artificial Sequence
tacacgacgctcttccgatctatcatgcttagccgccactccaccggcggc

SEQ ID NO: 258 - DNA, 52 bp, Artificial Sequence
tacacgacgctcttccgatctgatgcacatctgccgccactccaccggcggc

SEQ ID NO: 259 - DNA, 53 bp, Artificial Sequence
tacacgacgctcttccgatctcgattgctcgacgccgccactccaccggcggc

SEQ ID NO: 260 - DNA, 54 bp, Artificial Sequence
tacacgacgctcttccgatcttcgatagcaattcgccgccactccaccggcggc

SEQ ID NO: 261 - DNA, 55 bp, Artificial Sequence
tacacgacgctcttccgatctatcgatagttgcttgccgccactccaccggcggc

SEQ ID NO: 262 - DNA, 56 bp, Artificial Sequence
tacacgacgctcttccgatctgatcgatccagttaggccgccactccaccggcggc

SEQ ID NO: 263 - DNA, 57 bp, Artificial Sequence
tacacgacgctcttccgatctcgatcgatttgagcctgccgccactccaccggcggc

SEQ ID NO: 264 - DNA, 58 bp, Artificial Sequence
tacacgacgctcttccgatctacgatcgatacacgatcgccgccactccaccggcggc

SEQ ID NO: 265 - DNA, 59 bp, Artificial Sequence
tacacgacgctcttccgatcttacgatcgatggtccagagccgccactccaccggcggc

SEQ ID NO: 266 - DNA, 50 bp, Artificial Sequence
agacgtgtgctcttccgatcttaagtagagtcgccgtccagctcgaccag

SEQ ID NO: 267 - DNA, 51 bp, Artificial Sequence
agacgtgtgctcttccgatctatcatgcttatcgccgtccagctcgaccag

SEQ ID NO: 268 - DNA, 52 bp, Artificial Sequence
agacgtgtgctcttccgatctgatgcacatcttcgccgtccagctcgaccag

SEQ ID NO: 269 - DNA, 53 bp, Artificial Sequence
agacgtgtgctcttccgatctcgattgctcgactcgccgtccagctcgaccag

SEQ ID NO: 270 - DNA, 54 bp, Artificial Sequence
agacgtgtgctcttccgatcttcgatagcaattctcgccgtccagctcgaccag

SEQ ID NO: 271 - DNA, 55 bp, Artificial Sequence
agacgtgtgctcttccgatctatcgatagttgctttcgccgtccagctcgaccag

SEQ ID NO: 272 - DNA, 56 bp, Artificial Sequence
agacgtgtgctcttccgatctgatcgatccagttagtcgccgtccagctcgaccag

SEQ ID NO: 273 - DNA, 57 bp, Artificial Sequence
agacgtgtgctcttccgatctcgatcgatttgagccttcgccgtccagctcgaccag

SEQ ID NO: 274 - DNA, 58 bp, Artificial Sequence
agacgtgtgctcttccgatctacgatcgatacacgatctcgccgtccagctcgaccag

SEQ ID NO: 275 - DNA, 59 bp, Artificial Sequence
agacgtgtgctcttccgatcttacgatcgatggtccagatcgccgtccagctcgaccag

SEQ ID NO: 276 - DNA, 18 bp, Artificial Sequence
ggggaactcgggcaacct

SEQ ID NO: 277 - DNA, 19 bp, Artificial Sequence
gaatcggatctgccccgtg

SEQ ID NO: 278 - DNA, 19 bp, Artificial Sequence
catcgaggccaagctggaa

SEQ ID NO: 279 - DNA, 20 bp, Artificial Sequence
gtagtgaggagggagacccc

SEQ ID NO: 280 - DNA, 20 bp, Artificial Sequence
aagcctccttccttccccaa

SEQ ID NO: 281 - DNA, 21 bp, Artificial Sequence
atcgatacactccctagccca

SEQ ID NO: 282 - DNA, 22 bp, Artificial Sequence
acaaattcggtacatcctcgac

SEQ ID NO: 283 - DNA, 21 bp, Artificial Sequence
ttcagccatctttggaaggtt

SEQ ID NO: 284 - DNA, 20 bp, Artificial Sequence
acgccgcattgaccatctat

SEQ ID NO: 285 - DNA, 20 bp, Artificial Sequence
tagccaggaggttctcaaca

SEQ ID NO: 286 - DNA, 21 bp, Artificial Sequence
ggcatggactgtggtcatgag

SEQ ID NO: 287 - DNA, 20 bp, Artificial Sequence
tgcaccaccaactgcttagc

SEQ ID NO: 288 - DNA, 22 bp, Artificial Sequence
ccccgtaatgcagaagaagacc

SEQ ID NO: 289 - DNA, 21 bp, Artificial Sequence
gtccttcagcttcagcctctg

SEQ ID NO: 290 - DNA, 20 bp, Artificial Sequence
aacgcaacatgaaggtgctc

SEQ ID NO: 291 - DNA, 20 bp, Artificial Sequence
accttgacggtgactttggg

SEQ ID NO: 292 - DNA, 20 bp, Artificial Sequence
cagtgcaatgagggaccagt

SEQ ID NO: 293 - DNA, 24 bp, Artificial Sequence
aggaccataggtacatcttcagag

SEQ ID NO: 294 - DNA, 22 bp, Artificial Sequence
cgaacgagttgtatcacctgga

SEQ ID NO: 295 - DNA, 20 bp, Artificial Sequence
cgatggctgtccctcaaagt

SEQ ID NO: 296 - DNA, 23 bp, Artificial Sequence
agttgctcttttcactcaaggtc

SEQ ID NO: 297 - DNA, 21 bp, Artificial Sequence
ttctctctgagttcagacgct

SEQ ID NO: 298 - DNA, 52 bp, Artificial Sequence
tacacgacgctcttccgatcttaagtagagtggcacaggaggaaagagcatc

SEQ ID NO: 299 - DNA, 49 bp, Artificial Sequence
agacgtgtgctcttccgatcttaagtagaggcaccacctccatgccctc

SEQ ID NO: 300 - DNA, 49 bp, Artificial Sequence
tacacgacgctcttccgatcttaagtagagcatcgcagactgcggcaag

SEQ ID NO: 301 - DNA, 52 bp, Artificial Sequence
agacgtgtgctcttccgatcttaagtagagagtccatgggcctgtggaatgt

SEQ ID NO: 302 - DNA, 19 bp, Artificial Sequence
gaaaaactggcccgagagc

SEQ ID NO: 303 - DNA, 20 bp, Artificial Sequence
ctgagtctgggctgagggac

SEQ ID NO: 304 - DNA, 20 bp, Artificial Sequence
cgcttccaggtcaacaacac

SEQ ID NO: 305 - DNA, 19 bp, Artificial Sequence
ctcgcgtagatcagcaccg

SEQ ID NO: 306 - DNA, 21 bp, Artificial Sequence
cccctctgagtcaggaaacat

SEQ ID NO: 307 - DNA, 19 bp, Artificial Sequence
gaagatgacaggggccagg

SEQ ID NO: 308 - DNA, 19 bp, Artificial Sequence
tagcactggctggaatgag

SEQ ID NO: 309 - DNA, 21 bp, Artificial Sequence
gtttcggaggtaacctgtaag

SEQ ID NO: 310 - DNA, 20 bp, Artificial Sequence
tacagcaaccatgagtacaa

SEQ ID NO: 311 - DNA, 19 bp, Artificial Sequence
tcaggtgtttcacataggc

SEQ ID NO: 312 - DNA, 19 bp, Artificial Sequence
ctgcaaccatgagtgagaa

SEQ ID NO: 313 - DNA, 21 bp, Artificial Sequence
cctttgaggtgctttagatag

SEQ ID NO: 314 - DNA, 19 bp, Artificial Sequence
gccctgagaaaggagacat

SEQ ID NO: 315 - DNA, 24 bp, Artificial Sequence
ctgttctggaggtactctaggtat

SEQ ID NO: 316 - DNA, 18 bp, Artificial Sequence
tttgaagagggctgagaa

SEQ ID NO: 317 - DNA, 19 bp, Artificial Sequence
tgttctggatatttcatgg

SEQ ID NO: 318 - DNA, 20 bp, Artificial Sequence
catctgcctccccatattcc

SEQ ID NO: 319 - DNA, 22 bp, Artificial Sequence
tccatcctagctcatctccaaa

SEQ ID NO: 320 - DNA, 18 bp, Artificial Sequence
tgctccagaaggccagac

SEQ ID NO: 321 - DNA, 25 bp, Artificial Sequence
ttcataaatactactaaggcacagg

SEQ ID NO: 322 - DNA, 21 bp, Artificial Sequence
acagatgaagtgctccttcca

SEQ ID NO: 323 - DNA, 21 bp, Artificial Sequence
gtcggagattcgtagctggat

SEQ ID NO: 324 - DNA, 21 bp, Artificial Sequence
cattgtggccaaggagatctg

SEQ ID NO: 325 - DNA, 21 bp, Artificial Sequence
cttcggagtttgggtttgctt

SEQ ID NO: 326 - DNA, 20 bp, Artificial Sequence
catcacttgctgctgacacg

SEQ ID NO: 327 - DNA, 18 bp, Artificial Sequence
tgtggaatctgccgggag

SEQ ID NO: 328 - DNA, 18 bp, Artificial Sequence
ctgactctaagtggcatt

SEQ ID NO: 329 - DNA, 18 bp, Artificial Sequence
tgatggccttcgattctg

SEQ ID NO: 330 - DNA, 23 bp, Artificial Sequence
cggagtcaacggatttggtcgta

SEQ ID NO: 331 - DNA, 24 bp, Artificial Sequence
agccttctccatggtggtgaagac

SEQ ID NO: 332 - DNA, 2820 bp, Artificial Sequence
atggccgagatcaaggagaaaatctgcgactatctcttcaatgtgtctgactcctctgccctgaatttggctaaaaatattggccttaccaaggcccgagatataaatgctgtgctaattgacatggaaaggcagggggatgtctatagacaagggacaacccctcccatatggcatttgacagacaagaagcgagagaggatgcaaatcaagagaaatacgaacagtgttcctgaaaccgctccagctgcaatccctgagaccaaaagaaacgcagagttcctcacctgtaatatacccacatcaaatgcctcaaataacatggtaaccacagaaaaagtggagaatgggcaggaacctgtcataaagttagaaaacaggcaagaggccagaccagaaccagcaagactgaaaccacctgttcattacaatggcccctcaaaagcagggtatgttgactttgaaaatggccagtgggccacagatgacatcccagatgacttgaatagtatccgcgcagcaccaggtgagtttcgagccatcatggagatgccctccttctacagtcatggcttgccacggtgttcaccctacaagaaactgacagagtgccagctgaagaaccccatcagcgggctgttagaatatgcccagttcgctagtcaaacctgtgagttcaacatgatagagcagagtggaccaccccatgaacctcgatttaaattccaggttgtcatcaatggccgagagtttcccccagctgaagctggaagcaagaaagtggccaagcaggatgcagctatgaaagccatgacaattctgctagaggaagccaaagccaaggacagtggaaaatcagaagaatcatcccactattccacagagaaagaatcagagaagactgcagagtcccagacccccaccccttcagccacatccttcttttctgggaagagccccgtcaccacactgcttgagtgtatgcacaaattggggaactcctgcgaattccgtctcctgtccaaagaaggccctgcccatgaacccaagttccaatactgtgttgcagtgggagcccaaactttccccagtgtgagtgctcccagcaagaaagtggcaaagcagatggccgcagaggaagccatgaaggccctgcatggggaggcgaccaactccatggcttctgataaccagcctgaaggtatgatctcagagtcacttgataacttggaatccatgatgcccaacaaggtcaggaagattggcgagctcgtgagatacctgaacaccaaccctgtgggtggccttttggagtacgcccgctcccatggctttgctgctgaattcaagttggtcgaccagtccggacctcctcacgagcccaagttcgtttaccaagcaaaagttgggggtcgctggttcccagccgtctgcgcacacagcaagaagcaaggcaagcaggaagcagcagatgcggctctccgtgtcttgattggggagaacgagaaggcagaacgcatgggtttcacagaggtaaccccagtgacaggggccagtctcagaagaactatgctcctcctctcaaggtccccagaagcacagccaaagacactccctctcactggcagcaccttccatgaccagatagccatgctgagccaccggtgcttcaacactctgactaacagcttccagccctccttgctcggccgcaagattctggccgccatcattatgaaaaaagactctgaggacatgggtgtcgtcgtcagcttgggaacagggaatcgctgtgtaaaaggagattctctcagcctaaaaggagaaactgtcaatgactgccatgcagaaataatctcccggagaggcttcatcaggtttctctacagtgagttaatgaaatacaactcccagactgcgaaggatagtatatttgaacctgctaagggaggagaaaagctccaaataaaaaagactgtgtcattccatctgtatatcagcactgctccgtgtggagatggcgccctctttgacaagtcctgcagcgaccgtgctatggaaagcacagaatcccgccactaccctgtcttcgagaatcccaaacaaggaaagctccgcaccaaggtggagaacggagaaggcacaatccctgtggaatccagtgacattgtgcctacgtgggatggcattcggctcggggagagactccgtaccatgtcctgtagtgacaaaatcctacgctggaacgtgctgggcctgcaaggggcactgttgacccacttcctgcagcccatttatctcaaatctgtcacattgggttaccttttcagccaagggcatctgacccgtgctatttgctgtcgtgtgacaagagatgggagtgcatttgaggatggactacgacatccctttattgtcaaccaccccaaggttggcagagtcagcatatatgattccaaaaggcaatccgggaagactaaggagacaagcgtcaactggtgtctggctgatggctatgacctggagatcctggacggtaccagaggcactgtggatgggccacggaatgaattgtcccgggtctccaaaaagaacatttttcttctatttaagaagctctgctccttccgttaccgcagggatctactgagactctcctatggtgaggccaagaaagctgcccgtgactacgagacggccaagaactacttcaaaaaaggcctgaaggatatgggctatgggaactggattagcaaaccccaggaggaaaagaacttttatctctgcccagtagattacaaggatgacgacgataagtag

SEQ ID NO: 333 - DNA, 3705 bp, Artificial Sequence
atgaatccgcggcaggggtattccctcagcggatactacacccatccatttcaaggctatgagcacagacagctcagataccagcagcctgggccaggatcttcccccagtagtttcctgcttaagcaaatagaatttctcaaggggcagctcccagaagcaccggtgattggaaagcagacaccgtcactgccaccttccctcccaggactccggccaaggtttccagtactacttgcctccagtaccagaggcaggcaagtggacatcaggggtgtccccaggggcgtgcatctcggaagtcaggggctccagagagggttccagcatccttcaccacgtggcaggagtctgccacagagaggtgttgattgcctttcctcacatttccaggaactgagtatctaccaagatcaggaacaaaggatcttaaagttcctggaagagcttggggaagggaaggccaccacagcacatgatctgtctgggaaacttgggactccgaagaaagaaatcaatcgagttttatactccctggcaaagaagggcaagctacagaaagaggcaggaacaccccctttgtggaaaatcgcggtctccactcaggcttggaaccagcacagcggagtggtaagaccagacggtcatagccaaggagccccaaactcagacccgagtttggaaccggaagacagaaactccacatctgtctcagaagatcttcttgagccttttattgcagtctcagctcaggcttggaaccagcacagcggagtggtaagaccagacagtcatagccaaggatccccaaactcagacccaggtttggaacctgaagacagcaactccacatctgccttggaagatcctcttgagtttttagacatggccgagatcaaggagaaaatctgcgactatctcttcaatgtgtctgactcctctgccctgaatttggctaaaaatattggccttaccaaggcccgagatataaatgctgtgctaattgacatggaaaggcagggggatgtctatagacaagggacaacccctcccatatggcatttgacagacaagaagcgagagaggatgcaaatcaagagaaatacgaacagtgttcctgaaaccgctccagctgcaatccctgagaccaaaagaaacgcagagttcctcacctgtaatatacccacatcaaatgcctcaaataacatggtaaccacagaaaaagtggagaatgggcaggaacctgtcataaagttagaaaacaggcaagaggccagaccagaaccagcaagactgaaaccacctgttcattacaatggcccctcaaaagcagggtatgttgactttgaaaatggccagtgggccacagatgacatcccagatgacttgaatagtatccgcgcagcaccaggtgagtttcgagccatcatggagatgccctccttctacagtcatggcttgccacggtgttcaccctacaagaaactgacagagtgccagctgaagaaccccatcagcgggctgttagaatatgcccagttcgctagtcaaacctgtgagttcaacatgatagagcagagtggaccaccccatgaacctcgatttaaattccaggttgtcatcaatggccgagagtttcccccagctgaagctggaagcaagaaagtggccaagcaggatgcagctatgaaagccatgacaattctgctagaggaagccaaagccaaggacagtggaaaatcagaagaatcatcccactattccacagagaaagaatcagagaagactgcagagtcccagacccccaccccttcagccacatccttcttttctgggaagagccccgtcaccacactgcttgagtgtatgcacaaattggggaactcctgcgaattccgtctcctgtccaaagaaggccctgcccatgaacccaagttccaatactgtgttgcagtgggagcccaaactttccccagtgtgagtgctcccagcaagaaagtggcaaagcagatggccgcagaggaagccatgaaggccctgcatggggaggcgaccaactccatggcttctgataaccagcctgaaggtatgatctcagagtcacttgataacttggaatccatgatgcccaacaaggtcaggaagattggcgagctcgtgagatacctgaacaccaaccctgtgggtggccttttggagtacgcccgctcccatggctttgctgctgaattcaagttggtcgaccagtccggacctcctcacgagcccaagttcgtttaccaagcaaaagttgggggtcgctggttcccagccgtctgcgcacacagcaagaagcaaggcaagcaggaagcagcagatgcggctctccgtgtcttgattggggagaacgagaaggcagaacgcatgggtttcacagaggtaaccccagtgacaggggccagtctcagaagaactatgctcctcctctcaaggtccccagaagcacagccaaagacactccctctcactggcagcaccttccatgaccagatagccatgctgagccaccggtgcttcaacactctgactaacagcttccagccctccttgctcggccgcaagattctggccgccatcattatgaaaaaagactctgaggacatgggtgtcgtcgtcagcttgggaacagggaatcgctgtgtaaaaggagattctctcagcctaaaaggagaaactgtcaatgactgccatgcagaaataatctcccggagaggcttcatcaggtttctctacagtgagttaatgaaatacaactcccagactgcgaaggatagtatatttgaacctgctaagggaggagaaaagctccaaataaaaaagactgtgtcattccatctgtatatcagcactgctccgtgtggagatggcgccctctttgacaagtcctgcagcgaccgtgctatggaaagcacagaatcccgccactaccctgtcttcgagaatcccaaacaaggaaagctccgcaccaaggtggagaacggagaaggcacaatccctgtggaatccagtgacattgtgcctacgtgggatggcattcggctcggggagagactccgtaccatgtcctgtagtgacaaaatcctacgctggaacgtgctgggcctgcaaggggcactgttgacccacttcctgcagcccatttatctcaaatctgtcacattgggttaccttttcagccaagggcatctgacccgtgctatttgctgtcgtgtgacaagagatgggagtgcatttgaggatggactacgacatccctttattgtcaaccaccccaaggttggcagagtcagcatatatgattccaaaaggcaatccgggaagactaaggagacaagcgtcaactggtgtctggctgatggctatgacctggagatcctggacggtaccagaggcactgtggatgggccacggaatgaattgtcccgggtctccaaaaagaacatttttcttctatttaagaagctctgctccttccgttaccgcagggatctactgagactctcctatggtgaggccaagaaagctgcccgtgactacgagacggccaagaactacttcaaaaaaggcctgaaggatatgggctatgggaactggattagcaaaccccaggaggaaaagaacttttatctctgcccagtagattacaaggatgacgacgataagtag

SEQ ID NO: 334 - DNA, 2130 bp, Artificial Sequence
atggatatagaagatgaagaaaacatgagttccagcagcactgatgtgaaggaaaaccgcaatctggacaacgtgtcccccaaggatggcagcacacctgggcctggcgagggctctcagctctccaatgggggtggtggtggccccggcagaaagcggcccctggaggagggcagcaatggccactccaagtaccgcctgaagaaaaggaggaaaacaccagggcccgtcctccccaagaacgccctgatgcagctgaatgagatcaagcctggtttgcagtacacactcctgtcccagactgggcccgtgcacgcgcctttgtttgtcatgtctgtggaggtgaatggccaggtttttgagggctctggtcccacaaagaaaaaggcaaaactccatgctgctgagaaggccttgaggtctttcgttcagtttcctaatgcctctgaggcccacctggccatggggaggaccctgtctgtcaacacggacttcacatctgaccaggccgacttccctgacacgctcttcaatggttttgaaactcctgacaaggcggagcctcccttttacgtgggctccaatggggatgactccttcagttccagcggggacctcagcttgtctgcttccccggtgcctgccagcctagcccagcctcctctccctgccttaccaccattcccacccccgagtgggaagaatcccgtgatgatcttgaacgaactgcgcccaggactcaagtatgacttcctctccgagagcggggagagccatgccaagagcttcgtcatgtctgtggtcgtggatggtcagttctttgaaggctcggggagaaacaagaagcttgccaaggcccgggctgcgcagtctgccctggccgccatttttaacttgcacttggatcagacgccatctcgccagcctattcccagtgagggtcttcagctgcatttaccgcaggttttagctgacgctgtctcacgcctggtcctgggtaagtttggtgacctgaccgacaacttctcctcccctcacgctcgcagaaaagtgctggctggagtcgtcatgacaacaggcacagatgttaaagatgccaaggtgataagtgtttctacaggaacaaaatgtattaatggtgaatacatgagtgatcgtggccttgcattaaatgactgccatgcagaaataatatctcggagatccttgctcagatttctttatacacaacttgagctttacttaaataacaaagatgatcaaaaaagatccatctttcagaaatcagagcgaggggggtttaggctgaaggagaatgtccagtttcatctgtacatcagcacctctccctgtggagatgccagaatcttctcaccacatgagccaatcctggaagaaccagcagatagacacccaaatcgtaaagcaagaggacagctacggaccaaaatagagtctggtgaggggacgattccagtgcgctccaatgcgagcatccaaacgtgggacggggtgctgcaaggggagcggctgctcaccatgtcctgcagtgacaagattgcacgctggaacgtggtgggcatccagggatccctgctcagcattttcgtggagcccatttacttctcgagcatcatcctgggcagcctttaccacggggaccacctttccagggccatgtaccagcggatctccaacatagaggacctgccacctctctacaccctcaacaagcctttgctcagtggcatcagcaatgcagaagcacggcagccagggaaggcccccaacttcagtgtcaactggacggtaggcgactccgctattgaggtcatcaacgccacgactgggaaggatgagctgggccgcgcgtcccgcctgtgtaagcacgcgttgtactgtcgctggatgcgtgtgcacggcaaggttccctcccacttactacgctccaagattaccaaacccaacgtgtaccatgagtccaagctggcggcaaaggagtaccaggccgccaaggcgcgtctgttcacagccttcatcaaggcggggctgggggcctgggtggagaagcccaccgagcaggaccagttctcactcacgcccgattacaaggatgacgacgataagtag

SEQ ID NO: 335 - DNA, 4401 bp, Artificial Sequence
atgatgagctttgtgcaaaaggggagctggctacttctcgctctgcttcatcccactattattttggcacaacaggaagctgttgaaggaggatgttcccatcttggtcagtcctatgcggatagagatgtctggaagccagaaccatgccaaatatgtgtctgtgactcaggatccgttctctgcgatgacataatatgtgacgatcaagaattagactgccccaacccagaaattccatttggagaatgttgtgcagtttgcccacagcctccaactgctcctactcgccctcctaatggtcaaggacctcaaggccccaagggagatccaggccctcctggtattcctgggagaaatggtgaccctggtattccaggacaaccagggtcccctggttctcctggcccccctggaatctgtgaatcatgccctactggtcctcagaactattctccccagtatgattcatatgatgtcaagtctggagtagcagtaggaggactcgcaggctatcctggaccagctggccccccaggccctcccggtccccctggtacatctggtcatcctggttcccctggatctccaggataccaaggaccccctggtgaacctgggcaagctggtccttcaggccctccaggacctcctggtgctataggtccatctggtcctgctggaaaagatggagaatcaggtagacccggacgacctggagagcgaggattgcctggacctccaggtatcaaaggtccagctgggatacctggattccctggtatgaaaggacacagaggcttcgatggacgaaatggagaaaagggtgaaacaggtgctcctggattaaagggtgaaaatggtcttccaggcgaaaatggagctcctggacccatgggtccaagaggggctcctggtgagcgaggacggccaggacttcctggggctgcaggtgctcggggtaatgacggtgctcgaggcagtgatggtcaaccaggccctcctggtcctcctggaactgccggattccctggatcccctggtgctaagggtgaagttggacctgcagggtctcctggttcaaatggtgcccctggacaaagaggagaacctggacctcagggacacgctggtgctcaaggtcctcctggccctcctgggattaatggtagtcctggtggtaaaggcgaaatgggtcccgctggcattcctggagctcctggactgatgggagcccggggtcctccaggaccagccggtgctaatggtgctcctggactgcgaggtggtgcaggtgagcctggtaagaatggtgccaaaggagagcccggaccacgtggtgaacgcggtgaggctggtattccaggtgttccaggagctaaaggcgaagatggcaaggatggatcacctggagaacctggtgcaaatgggcttccaggagctgcaggagaaaggggtgcccctgggttccgaggacctgctggaccaaatggcatcccaggagaaaagggtcctgctggagagcgtggtgctccaggccctgcagggcccagaggagctgctggagaacctggcagagatggcgtccctggaggtccaggaatgaggggcatgcccggaagtccaggaggaccaggaagtgatgggaaaccagggcctcccggaagtcaaggagaaagtggtcgaccaggtcctcctgggccatctggtccccgaggtcagcctggtgtcatgggcttccccggtcctaaaggaaatgatggtgctcctggtaagaatggagaacgaggtggccctggaggacctggccctcagggtcctcctggaaagaatggtgaaactggacctcagggacccccagggcctactgggcctggtggtgacaaaggagacacaggaccccctggtccacaaggattacaaggcttgcctggtacaggtggtcctccaggagaaaatggaaaacctggggaaccaggtccaaagggtgatgccggtgcacctggagctccaggaggcaagggtgatgctggtgcccctggtgaacgtggacctcctggattggcaggggccccaggacttagaggtggagctggtccccctggtcccgaaggaggaaagggtgctgctggtcctcctgggccacctggtgctgctggtactcctggtctgcaaggaatgcctggagaaagaggaggtcttggaagtcctggtccaaagggtgacaagggtgaaccaggcggtccaggtgctgatggtgtcccagggaaagatggcccaaggggtcctactggtcctattggtcctcctggcccagctggccagcctggagataagggtgaaggtggtgcccccggacttccaggtatagctggacctcgtggtagccctggtgagagaggtgaaactggccctccaggacctgctggtttccctggtgctcctggacagaatggtgaacctggtggtaaaggagaaagaggggctccgggtgagaaaggtgaaggaggccctcctggagttgcaggaccccctggaggttctggacctgctggtcctcctggtccccaaggtgtcaaaggtgaacgtggcagtcctggtggacctggtgctgctggcttccctggtgctcgtggtcttcctggtcctcctggtagtaatggtaacccaggacccccaggtcccagcggttctccaggcaaggatgggcccccaggtcctgcgggtaacactggtgctcctggcagccctggagtgtctggaccaaaaggtgatgctggccaaccaggagagaagggatcgcctggtgcccagggcccaccaggagctccaggcccacttgggattgctgggatcactggagcacggggtcttgcaggaccaccaggcatgccaggtcctaggggaagccctggccctcagggtgtcaagggtgaaagtgggaaaccaggagctaacggtctcagtggagaacgtggtccccctggaccccagggtcttcctggtctggctggtacagctggtgaacctggaagagatggaaaccctggatcagatggtcttccaggccgagatggatctcctggtggcaagggtgatcgtggtgaaaatggctctcctggtgcccctggcgctcctggtcatccaggcccacctggtcctgtcggtccagctggaaagagtggtgacagaggagaaagtggccctgctggccctgctggtgctcccggtcctgctggttcccgaggtgctcctggtcctcaaggcccacgtggtgacaaaggtgaaacaggtgaacgtggagctgctggcatcaaaggacatcgaggattccctggtaatccaggtgccccaggttctccaggccctgctggtcagcagggtgcaatcggcagtccaggacctgcaggccccagaggacctgttggacccagtggacctcctggcaaagatggaaccagtggacatccaggtcccattggaccaccagggcctcgaggtaacagaggtgaaagaggatctgagggctccccaggccacccagggcaaccaggccctcctggacctcctggtgcccctggtccttgctgtggtggtgttggagccgctgccattgctgggattggaggtgaaaaagctggcggttttgccccgtattatggagatgaaccaatggatttcaaaatcaacaccgatgagattatgacttcactcaagtctgttaatggacaaatagaaagcctcattagtcctgatggttctcgtaaaaaccccgctagaaactgcagagacctgaaattctgccatcctgaactcaagagtggagaatactgggttgaccctaaccaaggatgcaaattggatgctatcaaggtattctgtaatatggaaactggggaaacatgcataagtgccaatcctttgaatgttccacggaaacactggtggacagattctagtgctgagaagaaacacgtttggtttggagagtccatggatggtggttttcagtttagctacggcaatcctgaacttcctgaagatgtccttgatgtgcagctggcattccttcgacttctctccagccgagcttcccagaacatcacatatcactgcaaaaatagcattgcatacatggatcaggccagtggaaatgtaaagaaggccctgaagctgatggggtcaaatgaaggtgaattcaaggctgaaggaaatagcaaattcacctacacagttctggaggatggttgcacgaaacacactggggaatggagcaaaacagtctttgaatatcgaacacgcaaggctgtgagactacctattgtagatattgcaccctatgacattggtggtcctgatcaagaatttggtgtggacgttggccctgtttgctttttataa

SEQ ID NO: 336 - DNA, 3117 bp, Artificial Sequence
atgacttcctcgctgcagcggccctggcgggtgccctggctaccatggaccatcctgctggtcagcgctgcggctgcttcgcagaatcaagaacggctatgtgcgtttaaagatccgtatcagcaagaccttgggataggtgagagtagaatctctcatgaaaatgggacaatattatgctcgaaaggtagcacctgctatggcctttgggagaaatcaaaaggggacataaatcttgtaaaacaaggatgttggtctcacattggagatccccaagagtgtcactatgaagaatgtgtagtaactaccactcctccctcaattcagaatggaacataccgtttctgctgttgtagcacagatttatgtaatgtcaactttactgagaattttccacctcctgacacaacaccactcagtccacctcattcatttaaccgagatgagacaataatcattgctttggcatcagtctctgtattagctgttttgatagttgccttatgctttggatacagaatgttgacaggagaccgtaaacaaggtcttcacagtatgaacatgatggaggcagcagcatccgaaccctctcttgatctagataatctgaaactgttggagctgattggccgaggtcgatatggagcagtatataaaggctccttggatgagcgtccagttgctgtaaaagtgttttcctttgcaaaccgtcagaattttatcaacgaaaagaacatttacagagtgcctttgatggaacatgacaacattgcccgctttatagttggagatgagagagtcactgcagatggacgcatggaatatttgcttgtgatggagtactatcccaatggatctttatgcaagtatttaagtctccacacaagtgactgggtaagctcttgccgtcttgctcattctgttactagaggactggcttatcttcacacagaattaccacgaggagatcattataaacctgcaatttcccatcgagatttaaacagcagaaatgtcctagtgaaaaatgatggaacctgtgttattagtgactttggactgtccatgaggctgactggaaatagactggtgcgcccaggggaggaagataatgcagccataagcgaggttggcactatcagatatatggcaccagaagtgctagaaggagctgtgaacttgagggactgtgaatcagctttgaaacaagtagacatgtatgctcttggactaatctattgggagatatttatgagatgtacagacctcttcccaggggaatccgtaccagagtaccagatggcttttcagacagaggttggaaaccatcccacttttgaggatatgcaggttctcgtgtctagggaaaaacagagacccaagttcccagaagcctggaaagaaaatagcctggcagtgaggtcactcaaggagacaatcgaagactgttgggaccaggatgcagaggctcggcttactgcacagtgtgctgaggaaaggatggctgaacttatgatgatttgggaaagaaacaaatctgtgagcccaacagtcaatccaatgtctactgctatgcagaatgaacgcaacctgtcacataataggcgtgtgccaaaaattggtccttatccagattattcttcctcctcatacattgaagactctatccatcatactgacagcatcgtgaagaatatttcctctgagcattctatgtccagcacacctttgactataggggaaaaaaaccgaaattcaattaactatgaacgacagcaagcacaagctcgaatccccagccctgaaacaagtgtcaccagcctctccaccaacacaacaaccacaaacaccacaggactcacgccaagtactggcatgactactatatctgagatgccatacccagatgaaacaaatctgcataccacaaatgttgcacagtcaattgggccaacccctgtctgcttacagctgacagaagaagacttggaaaccaacaagctagacccaaaagaagttgataagaacctcaaggaaagctctgatgagaatctcatggagcactctcttaaacagttcagtggcccagacccactgagcagtactagttctagcttgctttacccactcataaaacttgcagtagaagcaactggacagcaggacttcacacagactgcaaatggccaagcatgtttgattcctgatgttctgcctactcagatctatcctctccccaagcagcagaaccttcccaagagacctactagtttgcctttgaacaccaaaaattcaacaaaagagccccggctaaaatttggcagcaagcacaaatcaaacttgaaacaagtcgaaactggagttgccaagatgaatacaatcaatgcagcagaacctcatgtggtgacagtcaccatgaatggtgtggcaggtagaaaccacagtgttaactcccatgctgccacaacccaatatgccaatgggacagtactatctggccaaacaaccaacatagtgacacatagggcccaagaaatgttgcagaatcagtttattggtgaggacacccggctgaatattaattccagtcctgatgagcatgagcctttactgagacgagagcaacaagctggccatgatgaaggtgttctggatcgtcttgtggacaggagggaacggccactagaaggtggccgaactaattccaataacaacaacagcaatccatgttcagaacaagatgttcttgcacagggtgttccaagcacagcagcagatcctgggccatcaaagcccagaagagcacagaggcctaattctctggatctttcagccacaaatgtcctggatggcagcagtatacagataggtgagtcaacacaagatggcaaatcaggatcaggtgaaaagatcaagaaacgtgtgaaaactccctattctcttaagcggtggcgcccctccacctgggtcatctccactgaatcgctggactgtgaagtcaacaataatggcagtaacagggcagttcattccaaatccagcactgctgtttaccttgcagaaggaggcactgctacaaccatggtgtctaaagatataggaatgaactgtctgtga

SEQ ID NO: 337 - DNA, 3590 bp, Artificial Sequence
atgcctacagctgagagtgaagcaaaagtaaaaaccaaagttcgctttgaagaattgcttaagacccacagtgatctaatgcgtgaaaagaaaaaactgaagaaaaaacttgtcaggtctgaagaaaacatctcacctgacactattagaagcaatcttcactatatgaaagaaactacaagtgatgatcccgacactattagaagcaatcttccccatattaaagaaactacaagtgatgatgtaagtgctgctaacactaacaacctgaagaagagcacgagagtcactaaaaacaaattgaggaacacacagttagcaactgaaaatcctaatggtgatgctagtgtagaggaagacaaacaaggaaagccaaataaaaaggtgataaagacggtgccccagttgactacacaagacctgaaaccggaaactcctgagaataaggttgattctacacaccagaaaacacatacaaagccacagccaggcgttgatcatcagaaaagtgagaaggcaaatgagggaagagaagagactgatttagaagaggatgaagaattgatgcaagcatatcagtgccatgtaactgaagaaatggcaaaggagattaagaggaaaataagaaagaaactgaaagaacagttgacttactttccctcagatactttattccatgatgacaaactaagcagtgaaaaaaggaaaaagaaaaaggaagttccagtcttctctaaagctgaaacaagtacattgaccatctctggtgacacagttgaaggtgaacaaaagaaagaatcttcagttagatcagtttcttcagattctcatcaagatgatgaaataagctcaatggaacaaagcacagaagacagcatgcaagatgatacaaaacctaaaccaaaaaaaacaaaaaagaagactaaagcagttgcagataataatgaagatgttgatggtgatggtgttcatgaaataacaagccgagatagcccggtttatcccaaatgtttgcttgatgatgaccttgtcttgggagtttacattcaccgaactgatagacttaagtcagattttatgatttctcacccaatggtaaaaattcatgtggttgatgagcatactggtcaatatgtcaagaaagatgatagtggacggcctgtttcatcttactatgaaaaagagaatgtggattatattcttcctattatgacccagccatatgattttaaacagttaaaatcaagacttccagagtgggaagaacaaattgtatttaatgaaaattttccctatttgcttcgaggctctgatgagagtcctaaagtcatcctgttctttgagattcttgatttcttaagcgtggatgaaattaagaataattctgaggttcaaaaccaagaatgtggctttcggaaaattgcctgggcatttcttaagcttctgggagccaatggaaatgcaaacatcaactcaaaacttcgcttgcagctatattacccacctactaagcctcgatccccattaagtgttgttgaggcatttgaatggtggtcaaaatgtccaagaaatcattacccatcaacactgtacgtaactgtaagaggactgaaagttccagactgtataaagccatcttaccgctctatgatggctcttcaggaggaaaaaggtaaaccagtgcattgtgaacgtcaccatgagtcaagctcagtagacacagaacctggattagaagagtcaaaggaagtaataaagtggaaacgactccctgggcaggcttgccgtatcccaaacaaacacctcttctcactaaatgcaggagaacgaggatgtttttgtcttgatttctcccacaatggaagaatattagcagcagcttgtgccagccgggatggatatccaattattttatatgaaattccttctggacgtttcatgagagaattgtgtggccacctcaatatcatttatgatctttcctggtcaaaagatgatcactacatccttacttcatcatctgatggcactgccaggatatggaaaaatgaaataaacaatacaaatactttcagagttttacctcatccttcttttgtttacacggctaaattccatccagctgtaagagagctagtagttacaggatgctatgattccatgatacggatatggaaagttgagatgagagaagattctgccatattggtccgacagtttgacgttcacaaaagttttatcaactcactttgttttgatactgaaggtcatcatatgtattcaggagattgtacaggggtgattgttgtttggaatacctatgtcaagattaatgatttggaacattcagtgcaccactggactataaataaggaaattaaagaaactgagtttaagggaattccaataagttatttggagattcatcccaatggaaaacgtttgttaatccataccaaagacagtactttgagaattatggatctccggatattagtagcaaggaagtttgtaggagcagcaaattatcgggagaagattcatagtactttgactccatgtgggacttttctgtttgctggaagtgaggatggtatagtgtatgtttggaacccagaaacaggagaacaagtagccatgtattctgacttgccattcaagtcacccattcgagacatttcttatcatccatttgaaaatatggttgcattctgtgcatttgggcaaaatgagccaattcttctgtatatttacgatttccatgttgcccagcaggaggctgaaatgttcaaacgctacaatggaacatttccattacctggaatacaccaaagtcaagatgccctatgtacctgtccaaaactaccccatcaaggctcttttcagattgatgaatttgtccacactgaaagttcttcaacgaagatgcagctagtaaaacagaggcttgaaactgtcacagaggtgatacgttcctgtgctgcaaaagtcaacaaaaatctctcatttacttcaccaccagcagtttcctcacaacagtctaagttaaagcagtcaaacatgctgaccgctcaagagattctacatcagtttggtttcactcagaccgggattatcagcatagaaagaaagccttgtaaccatcaggtagatacagcaccaacggtagtggctctttatgactacacagcgaatcgatcagatgaactaaccatccatcgcggagacattatccgagtgtttttcaaagataatgaagactggtggtatggcagcataggaaagggacaggaaggttattttccagctaatcatgtggctagtgaaacactgtatcaagaactgcctcctgagataaaggagcgatcccctcctttaagccctgaggaaaaaactaaaatagaaaaatctccagctcctcaaaagcaatcaatcaataagaacaagtcccaggacttcagactaggctcagaatctatgacacattctgaaatgagaaaagaacagagccatgaggaccaaggacacataatggatacacggatgaggaagaacaagcaagcaggcagaaaagtcactctaatagagta

SEQ ID NO: 338 - DNA, 1677 bp, Artificial Sequence
atggctcaagattcagtagatctttcttgtgattatcagttttggatgcagaagctttctgtatgggatcaggcttccactttggaaacccagcaagacacctgtcttcacgtggctcagttccaggagttcctaaggaagatgtatgaagccttgaaagagatggattctaatacagtcattgaaagattccccacaattggtcaactgttggcaaaagcttgttggaatccttttattttagcatatgatgaaagccaaaaaattctaatatggtgcttatgttgtctaattaacaaagaaccacagaattctggacaatcaaaacttaactcctggatacagggtgtattatctcatatactttcagcactcagatttgataaagaagttgctcttttcactcaaggtcttgggtatgcacctatagattactatcctggtttgcttaaaaatatggttttatcattagcgtctgaactcagagagaatcatcttaatggatttaacactcaaaggcgaatggctcccgagcgagtggcgtccctgtcacgagtttgtgtcccacttattaccctgacagatgttgaccccctggtggaggctctcctcatctgtcatggacgtgaacctcaggaaatcctccagccagagttctttgaggctgtaaacgaggccattttgctgaagaagatttctctccccatgtcagctgtagtctgcctctggcttcggcaccttcccagccttgaaaaagcaatgctgcatctttttgaaaagctaatctccagtgagagaaattgtctgagaaggatcgaatgctttataaaagattcatcgctgcctcaagcagcctgccaccctgccatattccgggttgttgatgagatgttcaggtgtgcactcctggaaaccgatggggccctggaaatcatagccactattcaggtgtttacgcagtgctttgtagaagctctggagaaagcaagcaagcagctgcggtttgcactcaagacctactttccttacacttctccatctcttgccatggtgctgctgcaagaccctcaagatatccctcggggacactggctccagacactgaagcatatttctgaactgctcagagaagcagttgaagaccagactcatgggtcctgcggaggtccctttgagagctggttcctgttcattcacttcggaggatgggctgagatggtggcagagcaattactgatgtcggcagccgaaccccccacggccctgctgtggctcttggccttctactacggcccccgtgatgggaggcagcagagagcacagactatggtccaggtgaaggccgtgctgggccacctcctggcaatgtccagaagcagcagcctctcagcccaggacctgcagacggtagcaggacagggcacagacacagacctcagagctcctgcacaacagctgatcaggcaccttctcctcaacttcctgctctgggctcctggaggccacacgatcgcctgggatgtcatcaccctgatggctcacactgctgagataactcacgagatcattggctttcttgaccagaccttgtacagatggaatcgtcttggcattgaaagccctagatcagaaaaactggcccgagagctccttaaagagctgcgaactcaagtctag

SEQ ID NO: 339 - DNA, 3825 bp, Artificial Sequence
atgcctgagccggggaagaagccagtctcagcttttagcaagaagccacggtcagtggaagtggccgcaggcagccctgccgtgttcgaggccgagacagagcgggcaggagtgaaggtgcgctggcagcgcggaggcagtgacatcagcgccagcaacaagtacggcctggccacagagggcacacggcatacgctgacagtgcgggaagtgggccctgccgaccagggatcttacgcagtcattgctggctcctccaaggtcaagttcgacctcaaggtcatagaggcagagaaggcagagcccatgctggcccctgcccctgcccctgctgaggccactggagcccctggagaagccccggccccagccgctgagctgggagaaagtgccccaagtcccaaagggtcaagctcagcagctctcaatggtcctacccctggagcccccgatgaccccattggcctcttcgtgatgcggccacaggatggcgaggtgaccgtgggtggcagcatcaccttctcagcccgcgtggccggcgccagcctcctgaagccgcctgtggtcaagtggttcaagggcaaatgggtggacctgagcagcaaggtgggccagcacctgcagctgcacgacagctacgaccgcgccagcaaggtctatctgttcgagctgcacatcaccgatgcccagcctgccttcactggcagctaccgctgtgaggtgtccaccaaggacaaatttgactgctccaacttcaatctcactgtccacgaggccatgggcaccggagacctggacctcctatcagccttccgccgcacgagcctggctggaggtggtcggcggatcagtgatagccatgaggacactgggattctggacttcagctcactgctgaaaaagagagacagtttccggaccccgagggactcgaagctggaggcaccagcagaggaggacgtgtgggagatcctacggcaggcacccccatctgagtacgagcgcatcgccttccagtacggcgtcactgacctgcgcggcatgctaaagaggctcaagggcatgaggcgcgatgagaagaagagcacagcctttcagaagaagctggagccggcctaccaggtgagcaaaggccacaagatccggctgaccgtggaactggctgaccatgacgctgaggtcaaatggctcaagaatggccaggagatccagatgagcggcagcaagtacatctttgagtccatcggtgccaagcgtaccctgaccatcagccagtgctcattggcggacgacgcagcctaccagtgcgtggtgggtggcgagaagtgtagcacggagctctttgtgaaagagccccctgtgctcatcacgcgccccttggaggaccagctggtgatggtggggcagcgggtggagtttgagtgtgaagtatcggaggagggggcgcaagtcaaatggctgaaggacggggtggagctgacccgggaggagaccttcaaataccggttcaagaaggacgggcagagacaccacctgatcatcaacgaggccatgctggaggacgcggggcactatgcactgtgcactagcgggggccaggcgctggctgagctcattgtgcaggaaaagaagctggaggtgtaccagagcatcgcagacctgatggtgggcgcaaaggaccaggcggtgttcaaatgtgaggtctcagatgagaatgttcggggtgtgtggctgaagaatgggaaggagctggtgcccgacagccgcataaaggtgtcccacatcgggcgggtccacaaactgaccattgacgacgtcacacctgccgacgaggctgactacagctttgtgcccgagggcttcgcctgcaacctgtcagccaagctccacttcatggaggtcaagattgacttcgtacccaggcaggaacctcccaagatccacctggactgcccaggccgcataccagacaccattgtggttgtagctggaaataagctacgtctggacgtccctatctctggggaccctgctcccactgtgatctggcagaaggctatcacgcaggggaataaggccccagccaggccagccccagatgccccagaggacacaggtgacagcgatgagtgggtgtttgacaagaagctgctgtgtgagaccgagggccgggtccgcgtggagaccaccaaggaccgcagcatcttcacggtcgagggggcagagaaggaagatgagggcgtctacacggtcacagtgaagaaccctgtgggcgaggaccaggtcaacctcacagtcaaggtcatcgacgtgccagacgcacctgcggcccccaagatcagcaacgtgggagaggactcctgcacagtacagtgggagccgcctgcctacgatggcgggcagcccatcctgggctacatcctggagcgcaagaagaagaagagctaccggtggatgcggctgaacttcgacctgattcaggagctgagtcatgaagcgcggcgcatgatcgagggcgtggtgtacgagatgcgcgtctacgcggtcaacgccatcggcatgtccaggcccagccctgcctcccagcccttcatgcctatcggtccccccagcgaacccacccacctggcagtagaggacgtctctgacaccacggtctccctcaagtggcggcccccagagcgcgtgggagcaggaggcctggatggctacagcgtggagtactgcccagagggctgctcagagtgggtggctgccctgcaggggctgacagagcacacatcgatactggtgaaggacctgcccacgggggcccggctgcttttccgagtgcgggcacacaatatggcagggcctggagcccctgttaccaccacggagccggtgacagtgcaggagatcctgcaacggccacggcttcagctgcccaggcacctgcgccagaccattcagaagaaggtcggggagcctgtgaaccttctcatccctttccagggcaagccccggcctcaggtgacctggaccaaagaggggcagcccctggcaggcgaggaggtgagcatccgcaacagccccacagacaccatcctgttcatccgggccgctcgccgcgtgcattcaggcacttaccaggtgacggtgcgcattgagaacatggaggacaaggccacgctggtgctgcaggttgttgacaagccaagtcctccccaggatctccgggtgactgacgcctggggtcttaatgtggctctggagtggaagccaccccaggatgtcggcaacacggagctctgggggtacacagtgcagaaagccgacaagaagaccatggagtggttcaccgtcttggagcattaccgccgcacccactgcgtggtgccagagctcatcattggcaatggctactacttccgcgtcttcagccagaatatggttggctttagtgacagagcggccaccaccaaggagcccgtctttatccccagaccaggcatcacctatgagccacccaactataaggccctggacttctccgaggccccaagcttcacccagcccctggtgaaccgctcggtcatcgcgggctacactgctatgctctgctgtgctgtccggggtagccccaagcccaagatttcctggttcaagaatggcctggacctgggagaagacgcccgcttccgcatgttcagcaagcagggagtgttgactctggagattagaaagccctgcccctttgacgggggcatctatgtctgcagggccaccaacttacagggcgaggcacggtgtgagtgccgcctggaggtgcgagtgcctcagtga

SEQ ID NO: 340 - DNA, 1110 bp, Artificial Sequence
atgttgaagccatcattaccattcacatccctcttattcctgcagctgcccctgctgggagtggggctgaacacgacaattctgacgcccaatgggaatgaagacaccacagctgatttcttcctgaccactatgcccactgactccctcagtgtttccactctgcccctcccagaggttcagtgttttgtgttcaatgtcgagtacatgaattgcacttggaacagcagctctgagccccagcctaccaacctcactctgcattattggtacaagaactcggataatgataaagtccagaagtgcagccactatctattctctgaagaaatcacttctggctgtcagttgcaaaaaaaggagatccacctctaccaaacatttgttgttcagctccaggacccacgggaacccaggagacaggccacacagatgctaaaactgcagaatctggtgatcccctgggctccagagaacctaacacttcacaaactgagtgaatcccagctagaactgaactggaacaacagattcttgaaccactgtttggagcacttggtgcagtaccggactgactgggaccacagctggactgaacaatcagtggattatagacataagttctccttgcctagtgtggatgggcagaaacgctacacgtttcgtgttcggagccgctttaacccactctgtggaagtgctcagcattggagtgaatggagccacccaatccactgggggagcaatacttcaaaagagaatcctttcctgtttgcattggaagccgtggttatctctgttggctccatgggattgattatcagccttctctgtgtgtatttctggctggaacggacgatgccccgaattcccaccctgaagaacctagaggatcttgttactgaataccacgggaacttttcggcctggagtggtgtgtctaagggactggctgagagtctgcagccagactacagtgaacgactctgcctcgtcagtgagattcccccaaaaggaggggcccttggggaggggcctggggcctccccatgcaaccagcatagcccctactgggcccccccatgttacaccctaaagcctgaaacctga

SEQ ID NO: 341 - DNA, 151 bp, Artificial Sequence
gggtgatgggtgctggccaggacacccactgtatgattgctgtccaacacagccccagcctttgagacctctgcccagagttgttctccatccaacagggccatgagccccatgactgtgagtactggctttcgcagcaactgcacatggg

SEQ ID NO: 342 - DNA, 151 bp, Artificial Sequence
actacagttgctccgatatttaggctacgtcaataggcactaacttattggcgctggtgaacggacttcctctcgagtaccagaagatgactacaaaactcctttccattgcgagtatcggagtctggctcagtttggccagggaggcact

SEQ ID NO: 343 - RNA, 71 nt, Artificial Sequence
gucaaggcacucuugccuacgccaccagcuccaaccaccacaaguuuauauucagucauuuucagcaggcc